European Patent Application EP 4 574 167 A1, published June 25, 2025. Title: Toxoplasma gondii tachyzoite and bradyzoite native antigen inactivated vaccine. Applicant: SALUVET INNOVA, S.L. The sequence listing filed with the application follows.

SEQUENCE LISTING (96 sequences)

SEQ ID NO: 1 - protein, 769 aa, T. gondii
MRLQREAVFGLMFACGMWMWPSEVAGGGWSIVDALRKRYDTSRGGDANGVDTSGVEDVIQSESAIGAAEGCTNQLDICFLIDSSGSIGIQNFRLVKQFLHTFLMVLPIGPEEVNNAVVTYSTDVHLQWDLQSPNAVDKQLAAHAVLDMPYKKGSTNTSDGLKACKQILFTGSRPGREHVPKLVIGMTDGESDSDFRTVRAAKEIRELGGIVTVLAVGHYVKHSECRSMCGCSGTSDDDSPCPLYLRADWGQLATAIKPMLKEVCKTLPQDAICSDWSAWSPCSVSCGDGSQIRTRTEVSAPQPGTPTCPDCPAPMGRTCVEQGGLEEIRECSAGVCAVDAGCGVWGEWSAWSASCGNATRKRERTRYNDPPPQGAGRRCENQDPPVLQEQTEEATLAPCITIPPTPPEWAAWSDCTVTCGGGNRHRVRNALPPGLGSQNGESDESLVSKLWPGTDLRQEEACNTSPCPINATCGQFEEWSTCSVSCGGGLKTRSRNPWNEDQQHGGLSCEQQHPGGRTETITCNPQACPVDERPGEWAEWGECSVTCGDGVRERRRGKSLVEAKFGGRTIDQQNEALPEDLKIKNVEYEPCSYPACGASCTYVWSDWNKCVCPMGYQARHAAVKFDYRNKPCDLPTFETKACSCGETNPVPSEGTTPGAPGATGPEQPNQRPLPEGSDENETPTNEEGEQSKKESGSGIAGAIAGGVIGGLILLGAAGGASYHYYLSSSVGSPSAEIEYEADDGATKVVMEEEKETLVPVDDDSDMWME

SEQ ID NO: 2 - protein, 761 aa, T. gondii
MGSSHAIVACAALIVLLSTNARGLRVRKDKDVLLATSFLSHHGEYQNPTGTYNLIKEIRRVEAEIEDEVETLNRDRRLHRGHNKYADDDIRQGLKGEQDMGASENIPVAELEPQDLDREAKYPVRMLIVDKRSDDDDEETKTSFVETALHSDLAQRVVKELNGHVDVLRESGVVLVDLPAQTTDKQLQELIETARAQGTIVEPDHLVQSVNTSSKGSNDPLLDRLWGMDALNVKEAWDIITTGEPNMGGRRPLVCVLDTGIDYNHPDLRDNMEVNQAERDGTLGVDDDNNGEVDDIYGANMLSKENDPADDHSHGTHVAGTIGAHGNNGIGVAGVAWAPRLLPCKFLAYTGRGYSSDAVRCIDYCVKRGADIVNHSWGGSWPSEALREAVVRTANNGLIHIFAAGNDGVDIDQTAFYPAAFSTEADGLITVANVKGDPDHGGKRIIELDRSSNYGIQRVQVACPGMWILSTVPTSGSSQEPYAEKSGTSMAAPALSGIVALMLAVNPGLSTRQVREGLRQCSVQQPLLQGKVEWGSMPDAKRCVEYALTTHAEGRHKSFIREPSTETSTPPPPPPAQPTPQPQPHPPPQPETPPCAPSPPPPTPPCAPSPSPPTPPPGSPHKPEPQTPVYPEVPRSTRSPPPSPPPTESAPEAPPSDTPSCRVPPCSSSPRSGSQPKPPQDNTTTPKMPSLSSPPTEHSTAQPPKHENDAREQEPPTDEDDFSSVKGKKLGAYESDGSPRASSCAGAGVLGVFFMVVGLTV

SEQ ID NO: 3 - protein, 952 aa, T. gondii
MHPSGGQFVPTPQRHGPDLTKSWGLINRDFALRTREWAVSQRSLVFPVAVAAVRGETAPIAGRASQCPRLLVPFSWVLFLEQRPELSLTKVVFLLWNLYFVSLSPLRPFTGSLHPRPVVKMVNFSVEQMREIMGNPKNIRNMSVIAHVDHGKSTLTDSLVSKAGIISAKAAGDARFTDTRADEQERCITIKSTGISMYFEHDMEDGKGAQPYLINLIDSPGHVDFSSEVTAALRVTDGALVVVDTIEGVCVQTETVLRQALAERIRPVLHVNKVDRALLELQMDGEEIYQTFSRTIENVNVIISTYNDELMGDVQVYPEKGTVSFGSGLHGWAFTVERFSKIYAKKFDVPKEKMMERLWGNNFYNAKEKKWTKTQSENTRRAFCQFIMDPICTLFTSIMNDEKEKYTKMLGSLGIELKGDDRDLTGKALLKRVMQLWLPAGDTLLEMVVRHLPSPFAAQKYRVENLYEGPMDDEAAQGIRNCDPNAPLMMYVSKMVPTSDKGRFYAFGRVFSGTVATGQKVRIQGPRYVPGEKTDLYIKSIQRTVIMMGKYVEHVQDVPCGNTCCLVGVDQYLLKSGTLTTLDTAHNIADMKYSVSPVVRVAVKPKDNKELPKLVEGLKKLSKSDPLVVCTTEESGEHIIAGCGELHVEICLKDLRDEYAQIDFTVSDPVVSYRETVSAPSHMTCLSKSPNKHNRLYMVAEPFPDGLADAIEAGQVNARDDPKERANALAEKFDFDKNAALKIWCFGPETTGANMLIDTTQGVQYLNEIKEHCNSAFQWASKEGVLCEENMRGIRFNLTDVTMHADAIHRGAGQIMPTCRRVLYACQLASAPRLQEPMFLVDITCPQDAVGGIYSTLNTRRGHVFHEEQRSGTPLVEIKAYLPVAESFGFTTALRAATSGQAFPQCVFDHWSTLNGDPLEKGSKMEELVHNIRTRKNLKPEIPPFENYYDKL

SEQ ID NO: 4 - protein, 479 aa, T. gondii
MATVPMVSLSAARFTLSFLFFQLCLSRLFRPEGRNELEGPKDVDADVIRALDLASVFAFAEAVNNPPPLEGASVSPENATDPPETGGSRRWRTARYVLRRPFTHIRRVSSAVRRYISRGTSSLASSFAWKRRLRKLIRGMAKDLKQNRVRDAQQKPGSDAVASFVKTPHALLTSLGTPPAELANAVGLLLPVQHPVPMKSKVTGKSLLVSHAATVGVSSYGSVLLRCEGSGESASYFLEAFPVLRGSREASVSVRKQYLAAIKELRAASGVAQVGVVVDLLLLKRVRNTWCPRPHESHFAFPNVFLKRAVEGETLREVLLHIASTAATDTPGTGPAHDARVSLTEQVHKLARSAAELGSRGGKINIDTFFVTLDGIVHLQPVSLVESPPVHRGSAGLESPIAAELEEGEEKPSPEKRMTDDLALAIVLAQIWCPQRRFDDVAYELLLLHRFEREVTEEFFERCADPPEAVQVLVTMLAF

SEQ ID NO: 5 - protein, 333 aa, T. gondii
MLKTTPAFFLFLTWMFPRCDGFVLTHKNGTTDAYDSAVLSFLLTTEGVREGAAKSSGTEIPSTLACPSSSPLKTAKDKHDASLLGLVSSVPDSSILKPEFVGAGAALVAVTRSVKWTQLKQSLKALVDTGVKCKVNCKHNNKKLSKNTDFKDQQEFPQTSARILPTSDREPLIAGPQKVTEEDLQVLLFEIAHDCKMSAPQAAITKPLTILLAGIPGAHISKRPFEAAIPHFILQKEDTVDLLLTVDRSWCGKGLSHLVRYHVGYMSFNLEVNGRRLADDDTFEDDRLYRQVVLTTKFTAKSLGGTLKQVRSLTDIHKKTGKHGENRPHSSPF

SEQ ID NO: 6 - protein, 191 aa, T. gondii
MRTSRLLCAFGAVLLCWVPSWTAHAEEHFAVFSTCRTSFGRKRILVHSGDSVTIQCPGAIASNPQDVSKYVCPGEEPNCTDATKATYQTMFPIAPPDFQFWSGGDSKSNYGILKIPEVKDPVTISYSWQAAHSTFTGHAANSHLILDVNPKEEEVTRTVTSTVVVVSGCETQSLFTFLLVVASGIAMQQVL

SEQ ID NO: 7 - protein, 330 aa, T. gondii
MKLAAVSSAAFAAAFFPAVVNARKVGNPAAQPSVLVNEPVALAQLSTFLELVEVPCNSVHVQGVMTPNQMVKVTGAGWDNGVLEFYVTRPTKTGGDTSRSHLASIMCYSKDIDGVPSDKAGKCFLKNFSGEDSSEIDEKEVSLPIKSHNDAFMFVCSSNDGSALQCDVFALDNTNSSDGWKVNTVDLGVSVSPDLAFGLTADGVKVKKLYASSGLTAINDDPSLGCKAPPHSPPAGEEPSLPSPENSGSATPAEESPSESESVPSLPLSQIPSEVPLSQESPVPPQDGENPDSPQNEDNSMQEVENSASQSDIEAQRQAENGRLPSDDEA

SEQ ID NO: 8 - protein, 314 aa, T. gondii
MAGPKGKSDKRKTYFSRLFALLEKYPRVLVVEADHVGSKQMADIRLALRGKAVVLMGKNTMIRTALKQKMSEMPQLEKLLPLVRLNVGFIFCIEDPAEVRRIVAENKVPAPARQGVFAPIDVFIPAGPTGMDPGSTSFFQALGIATKIVKGQIEIQNEVHLIKEGDKVTASAATLLQKLNIKPFEYGLAIQHVYDDGSVYKASVLDITDEVILEKFRAGTMNVAALSREVGFPTTASAPHSILEAFKFCTSLVLESDYSFPQMQRIKDILENPEAFAAVAAAAAPAAGAAAAAEAPKEEEPEEEEDDMGFSLFD

SEQ ID NO: 9 - protein, 1280 aa, T. gondii
MLDVPILCALLVLLLSSLPAGAGALCVSLHRVSPSCLHSWEGGGCGFSSVFPPGRFASDCSERRRLPQPSLTTENVSASLNSGSALSSPPRRLSDFVRMQPRLLQERLFTDLSFLSRPRQTFSSSRLGVFSSPALSPLRSSSSATRVLLNFSRPARPRLCSRSPRHPSPSFCSSSIFPQSPSRSSLSSTWISLLLSDVRLASGAASLSSPWESFSLITSAARRPDSRAFARIPLVPLSIHSGKMAMTEEERRAKIEEISAKGKAKGWSGEAVRGAYLEFFEAQGHLIYPSSPVIPRGDNTLLFINAGMNQFKPIFLGQIDRSSPLSKLRRVADTQKCIRAGGKHNDLEDVGKDVYHHTFFEMLGNWSFGDYFKREAIAWAWQLLTEVYKIPKDRLYASYFGGDPRLPSCPPDEEARDIWLQYLPANRVLPFGAKENFWEMADTGPCGPCSEIHYDRIGGRDASSLVNADDPSVLEIWNLVFMQYNREKDGSLTPLPAPCVDTGMGLERVASVLQDKQSNYDTDLFTALFDKILELSPGLRPYGGKVGEEDKDMVDMAYRVLADHARCLTAAIADGAEPSNEGRGYVLRRILRRAVRYARQTLGMAEGNFPKLVPVVVSLLGETFPEMKKNEEKVVRILLKEEQQFSRTLDNGVERFKKVANSLQAKGQKVFPGGEAFTLYSTYGFPLDLTQLMAEEVGLQVDAEEFERKFDAHRAASENTSFKQGGAGAVYALPPDQRHLLAQSRKVPPTDDSAKYEWNVKDQAALMTQDAVEAAPIKAKVMAIWDGKRFAPEVTAVASPTGENLVAVILDKTCFYAEQGGQIGDVGRLVDLSSQAEFEVVDSQKSGDFILHIGSMSKGTLREGTELVPAVDYVRRFRLAQHHTGTHLLNFALREVLIRKLRSGGKASANGDKREDTNGIRICESCLNEKELEDGEDIQQKGSLVEVKRLRFDYAGEKPLENEDIIAVENVVKDCIAQARPVHYKEVPLEQAMKIPGLRAVFGEVYPDPVRVVSVGEDIESLVALADSSQPETPFASIELCGGTHLHNASQLSDFCILSEESVAKGVRRVVAAAGDAAFEARKELEELEEAFRSLASAPRELAALEKEVAKARGLLDGAGPLPLVGKRSLVKQLEQAQKALLELQKARSKELVKEAKKLGEELGTEHKTKPFLVLNLPQLLGDGKALDAASQTLHQAAPDLPFLLVTASAATGTAAIAFVPAACSQLHAASWLTACVGLLGGKGGGKGERAVGAAKEGAADKVDAAVAEATAFAEKKYGA

SEQ ID NO: 10 - protein, 290 aa, T. gondii
MSSHDLRLCRPRRQSKGSRQSPAFSAGRLCSSWGSLCVCRRVPRTKLGGSPAPRTAGIHRDSKCCATAMMPFPKRSLSLVCLLFCVVTAAGTLPRQPVADAFRLENQGVQDSHANSDAMQPSLGSATNHKATGTTSFVSVNENEEGMSQKAIIVFVVAISAMVICIGVVLVMWWMSSEREKKRRHVARDAERAPGLFFSEDEGPMSSDEKSAPKKPAGGNSPNTRDAGESISRERQIIEEDLGKVLVVDPVSGVMRSRQKWQRNGNSVPDKRMLAGTERTCRTGQQKFKK

SEQ ID NO: 11 - protein, 449 aa, T. gondii
MREIVHIQAGQCGNQIGAKFWEVISDEHGVDPTGTYTGDSDLQLERINVFYNEATGGRFVPRAILMDLEPGTMDSVRAGPFGQLFRPDNFVFGQTGAGNNWAKGHYTEGAELIDSVLDVVRKEAEGCDCLQGFQITHSLGGGTGSGMGTLLISKVREEYPDRIMETFSVFPSPKVSDTVVEPYNATLSVHQLVENADEVQVIDNEALYDICFRTLKLTTPTYGDLNHLVSAAMSGVTCSLRFPGQLNSDLRKLAVNLIPFPRLHFFLIGFAPLTSRGSQQYRALTVPELTQQMFDAKNMMCASDPRHGRYLTACALFRGRMSTKEVDEQMLNVQNKNSSYFVEWIPNNMKSAVCDIPPKGLKMSVTFVGNSTAIQEMFKRVSEQFTAMFRRKAFLHWYTGEGMDEMEFTEAESNMNDLVSEYQQYQDATAEEEGEFDDEDGGMDAEGEA

SEQ ID NO: 12 - protein, 300 aa, T. gondii
MKSGSCPFTFSPTLSHPLEIAWRARPLQWPEIERQPEPAAPCGALYPASRVLSFSPTMRAIRSVVGLPVMGAAVFLGLLSGELPNSSVLPVPEVASTPFLLSVAADGDGGKNYAEVAKVEALTNMISTPIELFVKDVWQQLFHKSGKPVWENMLFKFGSMIRHRAAHKATLVIMWELRHFLYGTAKVNPSAWKKLETKFETYLREWWMTVPEDPWAALHAGAWKSLLKLYNEDLEPLLRGSPKLKDLESILFDSKLATIRRWTDEAHIEVMKGRTSNMVPRLEALSAKMAVKQKAMQGKQ

SEQ ID NO: 13 - protein, 970 aa, T. gondii
MVTLSATTMNATVSPCRISGGVSSRLCGWGVLSFLLASVITVQVSRAGEEKEEPKAVVRLDYKPPNFYLEDIVLDFNLDDEDTTVEALLTLYRRAGTEPMNLVLDGDESVILKSISLATTSSPSLRGQGRVTFTELDGQMPTDSQFQFRIVDGNLMVSKFLLPREAEVRFYIRTLVSINPKANLALFGLYKAGDIFVTLNEPSGFRRITYGVDRPDVLATYTVTVTAPRHLPILLSNGDKVLSGYAGENRHFAKFVDPFPKPSYLFALVAGDFASVSGEFVTMSGRSVTVTIYAQHHQRNQLQWALRSLLRAMRWDEETFGREYQYSEFRVLCVEVFNPGAMENTSLNIFTCSLLLADPKLTTDADHRLIVDVVSHEYFHNWTGNRVTVQDWFQLTLKEGLTMFRNNSFTEETTSRAMKRIGDVADILSIQFREDSGPFAHPIRPETYKSIENLYTRTVYLKGAEVNRMYRTMLGPKGFRRGMDLYFKRHDGKAVTCDDLRAAMADANDKDLSQFERWYSQAGTPHVTVSSFIYDAAERKMHLTLKQHTPPTPGQDKKLPLQIPVAVGCIGKTSKRDVLSPPTQILELTEEEQAFVLVDVGEDCVLSVLRDFSAPVKLIQPLQTDEDLAFLVTYDSDNVNRWQAAQTLSRKVLLTRISEYQQRVEEIEEGRVSESDLFSKLPTQYVQTVRDIVIAPESSMGKDIKSLLLSLPTKAQLELAVDSIDPDAINAALASVRRDIVDALGEEMLQLYTELTLPAGTEESGADIEHWGRRALRNELLRFLTASFDQKSAKLASAHFDRAMVMSDKVAALTVLTEIPGQERDEAFERFRQEVAGNAVLMEKWMSLQAMSAAADTLERVAQLRQHSAFHPFIPGSAYSLFGTFSSSSPQFHSKTGAGYALVLDFLTMIDEHNSLVSSRIAGVAFANWKRFTSPRREMLKEVLKKLLKKEKLSVGLKEVLEKALAGEDD

SEQ ID NO: 14 - protein, 139 aa, T. gondii
MSQPTSPTVSPGTPLNCGASERQLEVESSPMEGRVYTDNEIHSDGGHSVECPPPGSPIPQTTTFTSQAAPALQPRMMYPSTDALTIPAGHQQMMYFNPAAAGYTDGSHGYDPREGYPVVYPYVPMTLPIETKKKRGFCC

SEQ ID NO: 15 - protein, 542 aa, T. gondii [sequence omitted]

SEQ ID NO: 16 - protein, 329 aa, T. gondii
MAPALVQRRKKVAMIGSGMIGGTMGYLCALRELADVVLYDVVKGMPEGKALDLSHVTSVVDTNVSVRAEYSYEAALTGADCVIVTAGLTKVPGKPDSEWSRNDLLPFNSKIIREIGQNIKKYCPKTFIIVVTNPLDCMVKVMCEASGVPTNMICGMACMLDSGRFRRYVADALSVSPRDVQATVIGTHGDCMVPLVRYITVNGYPIQKFIKDGVVTEKQLEEIAEHTKVSGGEIVRFLGQGSAYYAPAASAVAMATSFLNDEKRVIPCSVYCNGEYGLKDMFIGLPAVIGGAGIERVIELELNEEEKKQFQKSVDDVMALNKAVAALQA

SEQ ID NO: 17 - protein, 336 aa, T. gondii
MSVSLHHFIISSGFLASMFPKAVRRAVTAGVFAAPTLMSFLRCGAMASDPPLVANQVVTCPDKKSTAAVILTPTENHFTLKCPKTALTEPPTLAYSPNRQICPAGTTSSCTSKAVTLSSLIPEAEDSWWTGDSASLDTAGIKLTVPIEKFPVTTQTFVVGCIKGDDAQSCMVTVTVQARASSVVNNVARCSYGANSTLGPVKLSAEGPTTMTLVCGKDGVKVPQDNNQYCSGTTLTGCNEKSFKDILPKLSENPWQGNASSDNGATLTINKEAFPAESKSVIIGCTGGSPEKHHCTVQLEFAGAAGSAKSSAGTASHVSIFAMVTGLIGSIAACVA

SEQ ID NO: 18 - protein, 372 aa, T. gondii
MATRASLARQKTGAACLAVLTASPSVVAAKPWKRWVGVSVILASAFAVGVSAGPPYRYEPEKFTCRPKKGILSQWVSLLYQVQHNITFACEEATPVPTTLISEEHGLMVCAESMTPEECEANPAPLSAFLPGATKEWVTGDSVLTGLKISVPESQYPANAKSFRVGCRHNTKTGNTCMLTIHVEPRDPAVERQEARCSYTENSTLPKIFVTKDSNTMTLACGPHGAPMPESYTENYCSTPDTCDEKPFTSVIPGYLSKWFFGDPKSPLGAMLRIPPEQIPSSPQIIYLGCTGPTDGEGPKYNCTVPVQLGGEDPSEGSRPGGGSGGGKRGGGQGGGGGLAGSDSRQGSARHSLPSGMALSASALLAMTALAY

SEQ ID NO: 19 - protein, 112 aa, T. gondii
MPTKRRNGGRAKHGRGHSAVVRCSNCGRSCPKDKAIKRFNVRNIVDASSQRDLREASVYNTYTLPKLYIKQCYCVSCAIHSRVVRVRSVEQRKVRENPQRRPQGGQQGQGNN

SEQ ID NO: 20 - protein, 353 aa, T. gondii
MTHPNPLQTRFSRSASLVSRMPLVRLFFTIAAPLLFSPSPCPFLPLKTHCLAIQLGKPQGSPPASQKEAIRDTGVSHQKGEPSDSSSEPKPQGTVAETPGAASAAAAEVGRPSRSSAGPGKKKRGPSLFTEETMGPSKRHPCLKTLAAAVERFQAQHLTGRDAAKAFVDAIQECGIQVVASDYDRTAISVHSGGSARRDDLSVLGALTPDFKLLGEELTRRNIPIYFVTFSDKGENRGDRIAAGPLVEATLKASNANFEAQGVFGYYPPFYSEPEDYAPLGLSAPMPTDKSFHIQQVSKASGVPEDKILLLDDDRANCVNFCRSGGAAIHVSGHEGFDFGAVRVVVKPSLIMQ

SEQ ID NO: 21 - protein, 398 aa, T. gondii
MGGGGGGALNKLFPGYKDKIWMKVPVQWRQQMIQHWNKSYEKQVYSESVALNRTFQARNQLVLDRLKPSGAYRLPAVDYKRQLSRGTLVEGADFYLPTAQEQQRLARHFEPYSEQEQEERRKFRFQSISVYLAVALGASFVHDYFYQRRPVAWCLEKEPPHPPSYPFWFKSLFHSHDIPSVRRGYEVYRKVCATCHSMEQLHFRHLVGEVLPEKRVKQIAAEYDVTDGPNDQGEMYTRPGILGDAFPSPYPNEEAARYANGGAYPPDLSLITAARHFGPDYLMALLGGYRDPPEGVELRPGLYWNVWFPGNAIAMPPPLMDEMIDYEDGTPCNISQMSKDVVNFLTWATEPTADERKLYGLKCVSAIAIGTVLMTLWWRFYWAMYATRRIDFGKLKYL

SEQ ID NO: 22 - protein, 610 aa, T. gondii
MQKPVCLVVAMTPKRGIGINNGLPWPHLTTDFKHFSRVTKTTPEEASRLNGWLPRKFAKTGDSGLPSPSVGKRFNAVVMGRKTWESMPRKFRPLVDRLNIVVSSSLKEEDIAAEKPQAEGQQRVRVCASLPAALSLLEEEYKDSVDQIFVVGGAGLYEAALSLGVASHLYITRVAREFPCDVFFPAFPGDDILSNKSTAAQAAAPAESVFVPFCPELGREKDNEATYRPIFISKTFSDNGVPYDFVVLEKRRKTDDAATAEPSNAMSSLTSTRETTPVHGLQAPSSAAAIAPVLAWMDEEDRKKREQKELIRAVPHVHFRGHEEFQYLDLIADIINNGRTMDDRTGVGVISKFGCTMRYSLDQAFPLLTTKRVFWKGVLEELLWFIRGDTNANHLSEKGVKIWDKNVTREFLDSRNLPHREVGDIGPGYGFQWRHFGAAYKDMHTDYTGQGVDQLKNVIQMLRTNPTDRRMLMTAWNPAALDEMALPPCHLLCQFYVNDQKELSCIMYQRSCDVGLGVPFNIASYSLLTLMVAHVCNLKPKEFIHFMGNTHVYTNHVEALKEQLRREPRPFPIVNILNKERIKEIDDFTAEDFEVVGYVPHGRIQMEMAV

SEQ ID NO: 23 - protein, 588 aa, T. gondii
MCGILAILMSSLSRDQLRQLALERSRLSVFYRGGLDQECMGKSLWLRHRGPDSNGVHVQEYSTTLCNALAHERLAIVDPATGKQPLCDASGTFVCVANGEIYNHVELTKTLLPPEEVAKWKTASDCQPLPSLFKFHGPSICDKLDGIFSFVISNGATGEFIAARDPLGVCSLYVGYASDGSIWFASELKALTRDCEQVTVFPPGHFYLSTMNEGKGGFQRYYNPSWWGVDKPLPTYRCDLGQLREALEAAVRKRLMCDVPFGLMLSGGVDSSIIAAIAAKEFQKMSATEKGSHIWTNQIHAFSIGLKDGPDRKFAKMVADMLGTVHHEFTFELEEGLDALDDVIYMIETYDITTVRASVPMYLLCRMIKSLGVKVVLTGEGADEVFGGYLYFHSAPNREAFHRELQNKLNLVHFYDCLRANKTSMAWGVEARVPFLDRGFLDFAMSIDPEDKMCTNGRMEKQILRDAFKGYLPDEVLYRQKEQFSDGVGYAWIDHLKSYAEKKVTDTMMRNAKLLFPTNTPVTKEGYLYRAIFAKHYNKGSAARTVHTGPSIACSTAAALEWNEKFQECIDQSGRSVDVHQFHQGHRD

SEQ ID NO: 24 - protein, 269 aa, T. gondii
MALPLRVSATVFVVFAVFGVARAMNGPLSYHPSSYGASYPNPSNPLHGMPKPENPVRPPPPGFHPSVIPNPPYPLGTPAGMPQPEVPPLQHPPPTGSPPAAAPQPPYPVGTPGMPQPEIPPVHRPPPPGFRPEVAPVPPYPVGTPTGMPQPEIPAVHHPFPYVTTTTTAAPRVLVYKIPYGGAAPPRAPPVPPRMGPSDISTHVRGAIRRQPATATTTTTTRNVLLRTAILAAAAATLIALFRQRPLFTEGVRMFPDFQYRFTVQTTQN

SEQ ID NO: 25 - protein, 588 aa, T. gondii
MSKPFFPQVWVSCTGGVLNLRRHWLRVGNMSRAFAPTVLFVLLNVGGSLWVPRTLPVSAFQDAVAPHHPCIGRPCDQVASVVAVPPANNLGFKREPSVGSPGHFSFLQAVGGVGGPPYAGDGSPLLASRLDWQFLQQWHTDEDENARDGFVAALSRVTRLSQILEDCNMEMVLLLDRVFSRSPRITLSAVEPRTHRRRTLKLKIRSVAGTGGYNIVVKAFVIKSWFFRLGHWLGSLGRQRNTARAPGGETGQQTGTSGRRSSRSRGQSGREEGRREPQMVSLRIRVGGAPDCQVANEMQAAEVVQKCVSEADRIMHVFPEDVTPDVLVSRFRFAVPLYSGRIRHRSALLGQSRGYALLNYMDVLPPMLCDLFAAQSVVQPSMTRAIAKQLLELVAHLQALGVVHSDLKPENVLVDEAGNLFLADFDKAHKVGSRVRCSSLPHSLFADPQTVICRETTPDQEVTLAFSQDAWALGMLMYDTFCRNWPFMGMDYNNDSDTSNTIVLAGLLDRAAAVDTRAPIDWIGCDNPRVESEIKDLISRLLDIDPENRLDVLSFYMHSDFFNEGRNEANRSPPQRGAPILPLRESIV

SEQ ID NO: 26 - protein, 1410 aa, T. gondii
MVRHWRSPTFSWSPSVHFLLTSLAVFFLFSFFSPRFLDSSAATVQDAEEVERRRAPDNSPGVEASDALREGDRKPLSCEEDGRQPCTVSDYRVGLTDLQPLLQRVQALPSGVNLADVSEAATWISRPNSGSGGNCEGEADCAGEKTRAPFSADTVHGLTLPGPSQTTSTLSEETVAPGKGTFQMGVDPFSTVHGRGLSSGYDGVYLSNSGEDMSIERSFPDVVDEPGTPTSLPLHWFHPLYHFYPPEAFREEDSRSTSSKRTSAPLVWGARFLSPSRAGPRKSKASSAKHAGAVPASETRRPSHDEWLEPLEEREGGAREKKLRLSQSAEKTSSSIRSQSRFESQGTSRSSAAAHSSLVPSSLVSRIPSASQALHMQAPVDSSSLSHPRPVEVQGDLPAAVSESHAGDKAESPTLCLGRKAVVDSRSSQSRSASAEPSPERPAKTLSEPGSPDLASQSVVASDSRDECTGGNSSCVTSTPAAAVPAVQLPVSSFYPVVFHSSQTLAAVTEVSDLRRLGEDPLFDAEAVRHQEVCGGLFQWKRPMKASSSSDLACVWDRFADAFERTIPPRTPLPFRPGGFTYRTVDTVSRWYSRINSSSVPEVKSEQHREKAEASPSSPNQDAETLEPLSSRGTIHRSDSSSESSLSHESDAGVVAGSPHTPTPEKAKAVRRTTRSESPTGILGRSHAFLSKASRLISKRLTSFTWGLVQRLVTVLKNQQREGALMNLGKAINSMLESEGVTDTRAIESALFLPLGCKSHLHYSELYTEGYDVSPTDPTSWPDSPFFAWLIQDRARGEMLLPSNLPHHLTVTVSPRLPDDVEDKASRLRLYEMWHTIWFLIAEVSRSDYVWPWVKHKDVNQFFPWWTVTTVALHRVTEHRPVRYATGVWRFKNIDPETLEVIPQPDGSESNPFEVLPPPRSHLVEMQPGDNLATSGGDDQNPWGFLAEGLYANMAAAEQSANSRDDEDNAVKPKTFTYRGKSLSIYPDLCGEDATFSYLYDAPFAMLFTPSNLLERIRTRLHGRESDHPRWRQPRRTASRTSRQRKSRETVQGNLVDAIWIFKPTTMPKMWLANRMAKPFEPELSLSNHPEALVHRGYGLLFRTSYRPRMEQFISQLTSPQRPSSPLFPSSSLRGRDAMWLAYQHRSRAHPFTLVFAGHSQGGVAAEMSAFFVAKAMKDAIDNGTVRVYVIVFGTPSWCTQKMYEEFRETGLVIHEVASSVDPVPFLFTSTGFVADRKMVTLNLEDLYKVSFRHPFPFDGSLWKSPRKKTDKKTRLISATLGIRPLLDPTLSFTLTHSHVYAASLGLLSQRYPHIGWASFLGYPLVPPEVQTVPSHTPEGMRGLQEGHRLLLMGAGVEPPKSSSAAARGLSLLRSLRLRKRSREPDEGEEPPKKRRVVDKTLPEHDADRQ

SEQ ID NO: 27 - protein, 707 aa, T. gondii
MKVTTKGLAFALALLFCTRCATARYMSFEEAQKASEAAKRQIATLPSPDSTLSNPGSKHRNRGGSPAAGQPSQSTLQPEQAAAEVGLGAGGSTQGQGRTGGSAGAREERRSPSPQSAYPATSSASLRGYQTQLSPSHLPPRSSGPGGWFPTESIFTPWSSPPQPLTQRKPSLSGVVVTEFQEPQEQYGAASSLASSPKRYVSGASSSALSGKAVPTPASLGQENPLFPVQSATLDSGIQSPAQERRGSPQRQIAMSTENPADSGASQLASSVSSYVAVQTPHVKRSERIRRVRLSEEGLEEVQQLKAAAAQLLVAVPDYEAMRAVLQEAVLSEQRVATRKRKRKQPPGAVESAVDEVFPPNERVMMINANGVPIALYNRGHLGSGHFGAVIKASLDDGTLYAAKVPYSQIVPNADATSAELEAEISSARAELVKTIRQELDVRDKLVAKGLTLTETAEQYGLPLCQMTLTLPENKATVVRRGSRLVVVSKEVMLLPLIDGSPSNSLVQSQPPFLFQRAVAREAIIALAKLHELGFAHGDVKLNNMMIDVHGFGHMLDMGSVRPVDSCVSEEDKYYLRLWAPELAKSQHTSQQTCLKRGALDVWALGLAIFEFVCFNRLPYSLSNLPSSLWSRVEHLSRLRLSDFSAKDCNESDPAVMGIVAQFLNPNPEERPELPKFVSSYTFFRQAPGVTSHLTRIPTTELSSHRM

SEQ ID NO: 28 - protein, 351 aa, T. gondii
MSGGNSNTPKKLPSEEGSDYGYPQKPQKYLPKSEQAEPDYSACCKGNDAYKGASHGTVQFSHPEEAQKYAGAAAGAETIQRGRERVAADRQPRAAGDVPARRLHLSDVDEAHRGQSPSRHPGYCVEELCTCGMHKCIPSRAPVPFTGSTQYRQEFVPKPLPPPTQVSQVTLPPSLPFEAESSYRTEFVAKPLPPPAKFSEVKLPPTLPFHGESAYRTDYVPKPLPEVAKPVEVKLPPTLPFNAQSCYRSEYVAKPLPPPVQTVEVKLPPSLPFEGSTHYRDEFQVKPLPPATKVTEVKLPPSLPFDATSMYRSDYVAKSNPICPVSKLPQYPAATYPQNHVFWDPDTKQWY

SEQ ID NO: 29 - protein, 306 aa, T. gondii
MKLDVRVINLEDDSKQTVTVESWETVKTVKNLIEQKTGILESEQHYYLGVQLIEDSMPADQLRKKAKAEDRVPPDDSDGVHVVEVKMYTGKAPIDFDDSFFKDIIKKLQTHEQIMKHISVRVHRKGDDAKYNFHLDISFLTVESLKEDLINRLGPSSLTGLNADNILMYIRQEQPGRPLEGLQIRDRFGTRSSMEIEVFPINPEVTVVCKVKKWGLKTEEEFNIRIQDHFLLDDLKQILVTRLRSSANPKILQRDYIVGNLKFKLNGISINSKKEAALKRKYGIPAGELWLRAFNLKEGSLVVIPL

SEQ ID NO: 30 - protein, 475 aa, T. gondii
MFRLLVPTYYSYSVPLRFPFCKIYRYSTSNKMVAIKDITARQILDSRGNPTVEVDLLTDGGCFRAAVPSGASTGIYEALELRDKDQTKFMGKGVMKAVENIHKIIKPALIGKDPCDQKGIDKLMVEELDGTKNEWGWCKSKLGANAILAVSMACCRAGAAAKGMPLYKYIATLAGNPTDKMVMPVPFFNVINGGSHAGNKVAMQEFMIAPVGASTIQEAIQIGAEVYQHLKVVIKKKYGLDATNVGDEGGFAPNISGATEALDLLMEAIKVSGHEGKVKIAADVAASEFFLQDDKVYDLDFKTPNNDKSQRKTGEELRNLYKDLCQKYPFVSIEDPFDQDDFHSYAQLTNEVGEKVQIVGDDLLVTNPTRIEKAVQEKACNGLLLKVNQIGTVSESIEACQLAQKNKWGVMVSHRSGETEDSFIADLVVGLRTGQIKTGAPCRSERLCKYNQLMRIEESLGSDCQYAGAGFRHPN

SEQ ID NO: 31 - protein, 187 aa, T. gondii
MSFSKTTSLASLALTGLFVVFKFALASTTETPAPIECTAGATKTVEAPSSGSVVFQCGDKLTISPSGEGDVFYGKECTDSRKLTTVLPGAVLKAKVEQPPKGPATYTLSYDGTPEKPQVLCYKCVAEAGAPAGRNNDGGSSAPTPKDCKLIVRVPGADGRVTSGFDPVSLTGKVLAPGLAGLLITFV

SEQ ID NO: 32 - protein, 152 aa, T. gondii
MTVPGMKFSLIPKANRKAIYEYLFKEGVIVVQKNGKIERHPEVPVPNLHVMMTLRSLQTKKFVEEKFNWQHNYYFLTNEGIEFLRTYLHLPPTVFPSTLTKKSTGRPTRGAGEGMGEGGDMNGDWRPRGGFGRGRGRMGDRPDRAERAPRYA

SEQ ID NO: 33 - protein, 383 aa, T. gondii
MDVRYQTRGAVAAVYVLFRTVVGAVLGLHCLKIVSAEVGLTHGIMSTEFEVELRGHNWVIDSGACLLGQPRNLVVDPVLDSEFMTPQKLLTDRTGPELCSWLEKIHRQHMEQKPAWLAAYQKFEKRFFLLRLLGMVGKPITFFPEFTVRIIVKHFSLWGDDRWGNAQPWIAATFEYAHPEGAGGELFLHIEKVFSMEFSGRVAKLVHILLNPSATFNQYVELHRRKSSGVPGDSGVSGIRRTLYERDLNISHFPTADTSQISHSLAPDILTLRFAKQDFWMEDGSCYILSRFVATSSIRGKTLCKIVSDYGHRESWMPFVGSRKKTVALAVTAADFFNTRRPSLVAHIKEGVKLEALDKTPVVLELVTDPVILRSYVEAARKA

SEQ ID NO: 34 - protein, 181 aa, T. gondii
MLRPTVRSSLLSLGLTVILYLALTGSADALASHLRSRHMEAGRRTMDTQNDVESAGRQSEPMEAADRQAEHPGAPTQSEMKEFQEEIKEGVEETKHEGDPEMTRLMVTEKQESKNFSKMAKSQSFSTRIEELGGSISFLTETGVTMIELPKTVSEHDMDQLLHDILAAGGVVGLDSEVKLA

SEQ ID NO: 35 - protein, 328 aa, T. gondii
MVSCKRLAASRRQCLFFNACLFCLFICTVQIRAIAGADPEKCDQDGSLLNLRVTGNSSVEFKCGGAVPNLHPNPGKTPPIVCENSSCTNEVPLNIPNATLVKDSSGKATFTVSDASVGATTVYLKCSSLANTAARVGAGQPGQEAEKEKTCIVQTSVWGPPIKGSKEYPTPDACKNGTLSLEVNSSKKSVTFACGDNETLSPELFDMVFSTKECTTSSTLAEHLSGASLVQHARTNAADDKKPAYTFSVTSLPTEEKTLCYQCTKKNAQMKGEAQNTCKVLIKVAKQETDTGSTTVAPPNESRAEHGQWNTALMISLITIPVVLMKML

SEQ ID NO: 36 - protein, 154 aa, T. gondii
MDTRGAGDLLIVTRWLGLIAGLLTLLQWCFILPSKAVSLSVDNGDFLKDINHDSWRFALFSFVPEVFIDIWTPFVMGMISVLCHFDFYPIDFNSKNFALFFVWNCLQALFGNLGYCGGIGIISGSFSLLVSLLSLICFVLDRNADARLHIDKRS

SEQ ID NO: 37 - protein, 221 aa, T. gondii
MGRRPARCYRYCKNKPYPKSRFCRGVPDAKIRIYDAGRKRADVDEFPGVAHLVSDEYEQISSEALEAARVCANKYMIKNCGKDNFHLRIRVHPFHVLRINKMLSCAGADRLQTGMRGAFGKPMGLVARVDIGQILMSIRTRESNVATAVTALRRAAFKFPGRQKVFVSNKWGFTKFTKVEYKKWQAEGRIVSDGVGAKWISTKGPLANTFPSAADITLPVA

SEQ ID NO: 38 - protein, 668 aa, T. gondii
MVVSCLCTAMSSALSQRNCILISCRLGRQRSRPPDAMKVYAPVFTCRRQFLYEKYTRRRCTTLGGLVALCVIFTAEAISRSQHPYGTSRSDLSPPATVDSTSYGMSILEAGGPSDEVAIPSDRLQTFRNASLDFDRAIRFPNQASVAESRQLRLMQMGECQNVYWGKKELISRITGKWKSALHPSCHESWFTYTSWSRTKTWRECAQALDNSYLYFSWVRRHNEADGACIWVKPSRRDVSKSDVEDCLVDVNPQKEVAVTGIVGSHHGCTTCEVGEWSETTCDSWCNDGVKGRFRELTGHTNSAHCSTSADANCDVCPNLWEVQRCSTAVECAQGIKPRVRFCPNEGREYTAEGWRACAERCQRKFNATNGDTANRDTFYKAECFRYSFNNDTSACILNPLHACPDAESASDVLWISGDVLSMPSADYTTVTWQEWQSWSSCSEVDPATGWKKRTRRPKTWGYRPDNVLSPLQWISVTPCASNVTLTRSELDLAMNPSAMCWVYSDFADWSTVSCEPRCGADRKKTRARAVRQMPVVQPDGRISESCASTEVSLEARQQTKDCPGFVSCGTGCVFGEWTAWSDCRCTAEGSTARTIRARELVSGSKESCTGLEEERKCEKVCEESIFSNGVTYAVAGGIGLVVVIGLGFIGRKFYRALPAERTRDNYL

SEQ ID NO: 39 - protein, 435 aa, T. gondii
MGAPSPVAAGVAARTKSPLLTVCVCGGGNSAHAVAAWLGQAHKNVRVNVLTRQPEKWQKEIRLETKICRWDHLGSITGRVNAVSSDPAEVVPEADLCLICAPANAHFPLLEKIRHHLKAGGIIGTAFGQGGFDWAMLKAFEAEDCRKNLGCYFALQNLPWLCRIIQYGSAVELIGPKDFLNATVVPGNMGQPVRLLISLLFDMPCRLLPNFMAITLSPSNQIIHPARYYSIFHKWDGKTPMKEDEIQWGLYNQFDEMSAEWLEKLSTELQAIKKALTARFPELDLSSVLPIKERVIKHYGADVKDTSTLQTVFATNRGYAGCRTPATKVEGGYVPAVNGRLFNEDIPFGLCVLKDIAEQMDVPTPSIDFMIEWHQKLMGKEFLKDGKLNPEMIHETSAPRAYGLTTPEEIVAPSLMAQNATLPFAHIDMLGRLLN

SEQ ID NO: 40 - protein, 456 aa, T. gondii
MGQALFLTVLLPVLFGVGPEAYGEASHSHSPASGRYIQQMLDQRCQEIAAELCQGGLRKMCVPSSRIVARNAVGITHQNTLEWRCFDTASLLESNQENNGVNCVDDCGHTIPCPGGVHRQNSNHATRHEILSKLVEEGVQRFCSPYQASANKYCNDKFPGTIARRSKGFGNNVEVAWRCYEKASLLYSVYAECASNCGTTWYCPGGRRGTSTELDKRHYTEEEGIRQAIGSVDSPCSEVEVCLPKDENPPVCLDESGQISRTGGGPPSQPPEMQQPADRSDERGGGKEQSPGGEAQPDHPTKGGNIDLPEKSTSPEKTPKTEIHGDSTKATLEEGQQLTLTFISTKLDVAVGSCHSLVANFLDGFLKFQTGSNSAFDVVEVEEPAGPAVLTIGLGHKGRLAVVLDYTRLNAALGSAAYVVEDSGCSSSEEVSFQGVGSGATLVVTTLGESPTAVSA

SEQ ID NO: 41 - protein, 525 aa, T. gondii
MTPSTCCFGVLFQSFRGNSASASEESCLGGGHPDGTTATVFRPKTFQALGLATDSDSEPEGRGGYQRLTESTRRKKKATGRIASLFGRGRGKGDEEASGDEGASGGKEQPLGPPSGIPRRRRFWQKEHVEPEDAVVRAFRRFLKYRVLDVETIEGAPSQLDRSSWTPSPPFFQPGEGSSKAVEYFVKQQTPALTDEMHKLLEVVDPVMPPGRPLQMSSPSSKRTTHFERGPMLRTDFFALTVDHQPFNMRIFPLPGGFEGEQKVEQYKKVMLNEQKVLSIFGVADGKKVSNAYHCYLPVEEVFFGKGQQVISLGPSLKMPSVVFLYPSASATLGQVAEAIKLAAQQQGTALVAQAAQLHITLQLIKLVAITTSKGILLRRLSLENFLLRGDGVVFLSGFSELVNEKEIFYETEDGTLVTQPPTRTSRGRRFTPADNSCDLGLVIFSLWCNGSPPEREPSGWVNLDFSSCESEVPVLVQQIICGLCRAHGYPPQNAFQTLGSHEFKQLRQLYRDVEQRAEVHLLVE

SEQ ID NO: 42 - protein, 463 aa, T. gondii
MCSIPPLRLLEVVDDLTCLVNSSQYSRWNFFTFTLPGFTLPMRKEFTSSCKGSFSNHPVPDHPCKLVVFFRPKMVVTAGADAYLKILEYGVKKTQLRIDRLLLQAFMAGIFVAMAGHCCTVLAGSYPTDPGDPLAVAKPTQKFIYGALFPVAFICIILTGAELFTGNTMTMLICYFQKRVTMLQLGVNWLGSLAGNWLGALFGAYFLSYLTGALGDEHVRQFLFRTCVNKISYGWGECFLRGVGCNTFVCLAVWAVIASENVAGKVLVMWFPIVAFCVGGYEHIIANMYTLQAGLMAGAPVAILDVIAFNFLPTLLGNIVGGCLLVGAVYAYNFYPTLSYTETTGAKVYVQEVGPVLDRRSSMQVSMTEREPDGQVVTEYEAVPFESFGGEYIVNKHATMAAPIPSRASSFLYPFQWQRQRSQSGNLSTHARLDLPNRPVEPPSDGLEVTPQSQTAESVAQQV

SEQ ID NO: 43 - protein, 411 aa, T. gondii
MPATLEEQAVVAPPGDQTAMSSLPFEDTAAGRQGDSVVKGAKDDTSKQPTAVAYATEDPPLPSEVKILRQQPVEANETTVERGSQVAREKLEKRAAGANCMIFLVVVWLVCTGVLLIFAFSPVNADLGITSMLLGVFIGIIGILSVSAKSKTGVQLYLVLGTVLLLLTVALWGYYIYILFRAARAAADIAADRASHWVSDTPPELLPDRYGSGAAELTSIEAVARQGGLLPDVPLDETVEPCRKGFEEYGANYFKSATSVFLGLSTRGQMCNYSHYDILDFKKWPVSCWRTCGFDHLAVDRVLDNTRLDDQKVMADFLAHLESLSPQETSACVLYSVRTACVAENTAYHYILLAVIAFLIFWTCCACMCCIPASLCVAGKYLSELKSYQKDKEAVERHTPPGADQIELAGA

SEQ ID NO: 44 - protein, 844 aa, T. gondii
MSFSLLVSCLRSPPFRPRFLWGSPRACRRVPEARSPSRLLFSAQRRLPFSPRGPRFSTMASGRRAEKGTVAALATEEKIGDPHFQVSENSPFLQKRLQVFEDLYEKQTRRLKEKPRREISIELPDGSKKSGTAFETSPYDVALQISKGLAEASLVAKVLYEQPSAESEAITAADDEEEEEAECPCGEHAEESPAEKWILYDMKRPLEGSCRLQLLKFDSDEAKHVFWHSSAHILGQAIEATFGAQLTVGPALTNGFYYDAYMGDAKVTEESYGRLEAAAAAVIKEDQAFRRLVCSKAEALELFADNPFKVQLIASKIPEHGLTTVYCCGSLVDLCRGPHIPSTGKVKAFQVIKHSASYWLGRQHLDSLQRVYGVSFPDKKLLKDYLKLLEEAKKRDHRVLGQNLHLFFFDTNVSPGSCFWLPDGAKVYNKLCMFMREEYRFRGFQEVISPNIFSCDLWKVSGHYQNYKENMYLFDVEGKEWGLKPMNCPGHCIMFKHLAPSYRQLPLRLADFGVLHRNELSGSLTGLTRVRRFQQDDAHIFCRLDQVKEEVADALNFLFFVYDQFGFSFELFLSTRPKKALGERAVWDSAEAALKAALEETGRPWQLNPGDGAFYGPKIDIRLWDALKRPHQCGTIQLDFQLPIRFNLQYRTQDEAVAGARDKAKEDKETGEKRTDSEHEQKEEEAFGVELPLRPGMARPVIIHRAILGSIERMCAVVIEHTGGKLPFWLSPKQCIVLPISDKVNDYAASVRDVLHSCGYEVGLDVSNNTVNKKIREAQLQQWNYLLVVGEKERADKTVTVRDRADPEHQKVLSMEDLLTLFEKQGMPNSRKTLTLDAWKKSQQ

SEQ ID NO: 45 - protein, 133 aa, T. gondii
MSSVEQKAREAFKLFDRNGDGELTHQEAVLAVRSCGIPLRIQELDLPEQVTYPQFRQWMMNRVARSDPLEDLIKLFAPFDRKNDGTISTEELAQVMKTLCSSMTEEDIDHLIKQADPNNSGNIKYAEFVHQCF

SEQ ID NO: 46 - protein, 472 aa, T. gondii
MELNLATQNASLGVTQATRAKSVSLNVMQTTTGSVMVGQEGWLEDGAAMTDNKHDCQLSVVQFVPLGSISVKQWCYFKVGYVYACLEYNGGLAKRQQGAEPPSLSVTALFITMAVPREISWTQSQREMRLQIPYGRLLTRQSTLFFVALLAVVLHDSFVAFHGHLCHFAEAAAHQGSCTSQGTSSPMQVCTCNVPEQGETSNHAVVVSAEKNQLMAKCAIGTVTLPVDLMEKQVVCPAGMTDPQSCVSPSGTIPFASLLSGDGASAVAWVGDEVNYAAVLQVPKQNLPPVDKEFIVGCTQEGKGHCLLHVTLSARASSKDSQTVTCAYGSASNADVHRVTVSPKDPTFTLDCSSDGIMQPASFTTSYCPATGPLQENCDEKYASILQGYSSSWWQVSQAGTSNKAVLTIPHDNFPEAQKKVLVGCKASTAIPNSTLCTVELTITSSSPSSAWFLSLSVTMTLAVAGAVSSLV

SEQ ID NO: 47 - protein, 446 aa, T. gondii
MACRQLLCSVQNLLFYFLPDIYCTDFDTMEQRLPIILLVLSVFFSSTPSAALSSHNGVPAYPSYAQASLSSNGEPRHRGIRGSFLMPVKPHANADDFASDDNYETLPSFVEAPVRDPRQVPGRGEAALGTEETPGQQPPVALGSAEGEGTSTNESASENSEDDTFHDALQELPEDGLEVPPPNAQELPPPNSQELPPPNSQELPPPNSQELPPPNAQELLPPTEQDLPPPTEQELPPPVGEGQGLQVPGEHGPQGPPDDDQQLLLEPTEEQQEGPQEPLPPPPPPTQGEQPEGQQPQGPVRQNFFRRALGAARSRFGGARRHVSGVFRRVRGGLNRIVGGVRSGFRRAREGVVGGVRRLTSAASQGLRRAGEGLRRGFTRVRGALRGRGRAADGASSVRERFGAASGRVRDAFSAGLTRLRRRGRTSGEEGRPLLGEGREQDDGSQ

SEQ ID NO: 48 - protein, 345 aa, T. gondii
MQGTWFSLFVVVMVSHLAFGGECSFGSYLADMAGLTGREDKEHHAAKKRYYHSMYGNKTPYPYADGQQGSPPPQGQLLIIQNPDGSFMIVDQQGVPQAPQAAGGPGSPMNGGYYMPAGVYTAQVVPGTPGHPVQAIPQQPLRTQATATYYHPAAAPPPGPSVFVFTPSSVQPGAEVTPGYSGLQLRQQSQYDYSYPGTTSTPTPPRPASYGYPAFPAFPRLPAFSDSVSVSTEDSGLTVVRDSSSSESTVTPADEAASESEEGDKTSRKSKVKKGVLTGLGVAATLAAAAAAAKAVKGFGGTRTSTAPAEAGKTELDDGYRPPPFNPRPSPYAELLKDLERMRKE

SEQ ID NO: 49 - protein, 511 aa, T. gondii
MQDPSGHGNRPRAALVQLQESWVCCAAPNSVFSADIRTVAQMFSPPCASRRPRVGFSQATLCAGRLPVSRFCSLLSFSDLPPRQDTRLFPSSFLNGVASEKTLAFLPYPLPRESVSGGSVQAPGAPVSGVRHDKFAFRLSPGSRPGSVSRFRFHRPSSSATAARHLQGESRPFASCPVTPEATPFPQPVPSSFFKMSRRKIGLIGGGNIGATLALLSAVKELGDVVMFDVVQDLPQGKCLDLYQLTPISGVDVRFEGSNDYSVLKDADVIIVTAGVPRKPGMSRDDLLAINAKIMGQVGEAIKQYCPNAFVICITNPLDVMVYILREKCGLPPHKVCGMAGVLDSARLRTFLSERLNVSVDDIHALVMGGHGDTMVPLPRFTTVGGIPLPELVKMGMISQQEVDDIVQRTRNGGGEIVSLLKTGSAFFAPAAAGVLMAEAYLKDRKRVLPCAAYLNGEYGVKDMYVGVPCVIGAGGVEKIVELDLTPEEKKMFERSVESVKTLLAAAPKSA

SEQ ID NO: 50 - protein, 619 aa, T. gondii
MSPSSRFRNLVSVDSSSQDFGKRSSLYASLLDSASVSSLPGICSAAEDRDVEDESWKDPSSSSHCAKTEGGACAFPRLNQVLSSLRDPMGVFSRAKRRRSLGKAVGLSTSVICVVALFGIVCLCLYGLVNFSFTSVETSPLDDPRNSPVMGELGNPQASTPSSARADTPARHDRQNQMFSPWSVQNEQFLGEDSDALPHAGPLFRSGVMVMPLRKMKSLRQIGWDKNTITVPDLQAHLVAALRMQEGLSKKDDGNLSGLSNGDDISIHDYMNSQYYTEIYVGSPGQKVRVVVDTGSSDLWVCSASCGILCMMHKTYNHGKSDTYHADGTPYHVQYASGPVGGFLSADDVALASLKTKNFLLAEAVDLKGLGTAFFFGKFDGILGMGFPSLATKGLKPFMQAAVEQNVVKNWVFAFYLASANGVDGELAIGGVDQERFIGDINFSPVVDSRYWMINTKGLKSDGDLIAPTTKMIIDSGTSLIVGPLDEVKRIATMMGAFSVPLMPEGMFFISCEKAKVLRDLQLEIEGQDYPIKIKDLLISASAAAGTPCLFGMMGLKALEGGRPTPQKNGFGIFPPSQLVASAKGPIGRTWILGDLFMRNVYTVFDYDNKQIGFARLKN

SEQ ID NO: 51 - protein, 330 aa, T. gondii
MNTGCLFLPATRHAAIQTICVVALARQVADPDALVFERDFLEFIRILSSTQTVFSSFGCPRSHVALLAQSVERVREANAVGLFSEFARRLGFPTSGDDAGCSCAFFVFTGRAMVWRVSIGCAVLATVLVAGHEPVASAPYKAYGIPAESTDTTSGDDVEEAFRKRSRGNVLKDAAKEEKKLPLFFIDVEDNKGQGRNSEKGATDDDVAVDKTKRSSPSAPCTRLAGKEKKYPCDRYVVKGKMSFLEAIGAFFLASVIHAAVSEQLRARSTGGDIWRPRLAGSVMQAALAATTLWMALRRRLPTFYLLQRRESSEEKKKAKENSTRAASAV

SEQ ID NO: 52 - protein, 364 aa, T. gondii
MAAAHSAAACRYSTFWPCLLRERQSGTSSVSFVYPSQFLSLSLLVILTGSFAQQSAGNQANSQSVTCESNASPLVLRITSKTNEVKFKCGTDLQLRENPAGSNKFWGNAACTKEVDASSVTFTSSPSPAKVAGNKGTEYSLALKNSSLPLSPFTVYFSCDPPSTTGVGETGKAKVPASATTCIVQVSVFSQTAVTVPETNKCKNGQVTVAVTSKSKSVTFGCSEGATLKPALLDHVFIEKATEKSGGASTGREEEVVLQDLVPNSSLVENAANTGNDTVGYTLSCPDLPSSPQNIFYKCVSPASAREQVGTQTECKVLINIEEKPEAETPATPEPSRGEQGVVLGSAFMIAFISCFALVAGNMF

SEQ ID NO: 53 - protein, 258 aa, T. gondii
MAGTSASREDSQSPAVRQRVGSASGGKSVQAASDSDLSHEQKWARELKVFLYVPNIIGYVRIALLLAAAFAWREAYTSLFFVSYVTSQCLDAVDGAAARRLGQVSIVGACLDQVVDRLSTCLLYVLNASVYPDFAFAFFIALFLDMGGHWVHFFAAAVVGAKSHKTMDPEVNAILSVYYRSRPVMFSAIVGFEGFFMCLLLLASPVFQASAASLSSALLVIVYVTSPLMIFKTLTNLLQGLYGARRLVACDIFGAPSS

SEQ ID NO: 54 - protein, 999 aa, T. gondii
MVPLSRMAMVSVAYFILGALVYGSANVFGEMQPRQLAKSSTDDPTIHDEGHGAAAPSTPRAGTELMTPHPLASRAKAVTSAIIQESKSTLFNTGHVTTTEHAPKNPGLLGKPVKQTEALQLASPEKGVTTMEPKAASQHADRSGNPAVKKSTSGAQQAAAQSGKVLTKLTPIEKNPAPLHRQPMTRATPVGPKPADPAGKAVKKAATGIPKPAAPGGKAVKVTPVARKPVAPKAAAPDGKAVKKATVVVPKPAAPSGKAVKKPVVSVPKPATLGGKAVKKPAAGVPKPAAPDGKAVRKPVVGVPKPAAPDGKAAKKPASGVPKPADPAGKAVKKAATGIPKPAAPGGKAVKVTPVARKPVAPKAAAPDGKAVKKATVVVPKPAAPSGKAVKKPVVSVPKPATLDGKAVRKPVVGVPKPAAPDGKAVKKPVVGVPKPAAPDDTGINKATLVTRKPEAPDVKVVKKATVVVPKPEAPDIKVMTDQTPTTPPSPPVRARAASATTIVTAPAPVPTRPVLTTTSTAATVTTIKTETPRAASRLQQDLNAFCTTQFQKLCSETIDGGRYCGVSGAVARFGPGGHDSDSQWRCYEESIMNTTTKGVQCMDDCGNQMQCVGAVSVKTVATPPLRALSAFISQRRWIYCSSFQRSADALCNFKRTGNVARYDPGRTRWMCFNPVDISLEGQSYCANNCGGFTPCAGGLSPGEIPTRTVYIIQQSDTAEAFAALHPCRHDEICIPSTVYPPACVKAHKIIAIQQLSKQQEAMDNYCQTEMDQMCRVGKWTTYCYQLWLSRMVSTEEDEEPKWRCYPFALLNFSDLSTCIDGCSNRVPCHGAPSPTSTLTTEFSKLKTIAENIAFCSPFQKAANDHCNKRYGEGWVARQDVTTDDWACFQTTKLPTYRWTGCVDNCGNTSLCAAGVPEQLHSAAAEAFVHPDPALERVVESVPSPCLTGESCTPTAMNPPYCSETRPNPQPAPLRDHTIRNALDCSKGAPLARRNPTSK

SEQ ID NO: 55 - protein, 571 aa, T. gondii
MRTSVALFFAAAGGISLVCAPQVSLAAPVQGTLGPDVADTAGEPVVLQVARGADSLPDSRGNIDEEGITEVATTGVPPQTQSSGRSFGQRVMSWFTSARNAIRRPRTDEQGAVPGPSQPIPSGTDSTPEGWETVQSGDVPPGEPEPKAPTRSPRQRARDMFGRVGRFFGGARRFVGRGWRRFTTGMAGVTDRVRGRLALRSSFEFRNEEAVGQSELASLASSMTVTAPEGEALEVAREAGLRSGASINLVSATTGEQVTVSLRAPLGIGEYTAVFSGFISGIDSELAVKAFLGKTTESMSVAETEARILKIVSLKDPVDAMHRLRLLAPIETLVYRGDGDSADQSEGRPVVLVPKASSSLVDVINFLRSGDASAFDDRAKKIVLLGATVQLIQLLAALHTRKVVHGKLEPKSVLLFSHGLLYLSDLGRARRHGERFTTSRPSRYGAPEVLEHPETPYTYSRDGYSLGIILFELWCGRLPFDLGTPGVDSSEKLENSHPATLYQTVRNLDQRLSFDVCPSDMPESVKTLIRKFLTRRRWTRLVPQAALRDANFRRTMQLLQETVQGNGETQL

SEQ ID NO: 56 - protein, 107 aa, T. gondii
MVKLRWKSASCTDRALQLMDVTLQRLEEEEENADKKGDNGTDRQRHIPTAINDLLYPSCIAVAVTPNVGEGACFRGMQCAQYSVLGKVYNIAVIMKPEEVLRSNGQE

SEQ ID NO: 57 - protein, 592 aa, T. gondii
MRGSVLVVTRTVDCRLSRFQGKCYFRQWPVSGTTRSHRTRGWYLTLLLPLQSAVMAHVLISSPSTVELDEETQVFTSLQNAALIPRDRRKTRTHVRLRRSRSGGTGSWKPLATRVLIVTFLVALAAVALRRYVLRTRSRSMSTVSQDSDISASPRETVLDDRARFRADDGGNEGEFAFPSSPVENVAAAVARLNHGSTTADEQPHRGGQADAALELLRPPTPSWGNQEAPEGVTGRITEAVAMPLPAIDSLGERPHNGEQASAALEPPGPATSPWGNEETPDGATGRITEAVAMPLPAIDSLGERPHNGEQASAALEPPGPATSPWGNEETPEGATGRITEAVAMPLPANDSFGERPHNGEQASAALEPPGPATSPWGNEETPDGATGRITEAVAMPLPAIDSLGERPHNGEQASAALEPPGPATSPWGNEETPEGATGRITEAVAMPLPANDSFGERPHNGEQASAALEPPGPATSPWGNEETPEGATGRITETVATSTVGSIAPAEQSHSGEQAGAVLEPPAAPKPWGILDAALEKVREEISKQQVQLHFAMRRGDSAEVDARKEMLLDLLKGRALLQSIPDEPGDGEIP

SEQ ID NO: 58 - protein, 3029 aa, T. gondii
MAARLRSLSLGRFCLLLLLATWSAWSAAGSSSASFSPEEESLVSHSRVPPEGKEASSAAAFEPTFRLVAFSPPSSSQQESVPVLRGRQPIAAVFSVPVVPLGSSLFSENASAPSEPRTPDAFRLSTNSAAKTVKGRGFWVTTSIFRFDPEEPWPADLEVYVHLNAELRSASGQLVTLPEDCGRGVAPQGGLKNHGMIAEKLDGEDERRSLATSNSRSACIVHLRTDSLRVSVASVTSEFASAVTDNEWKPVLGNSADPLAALFEVPRDGKVRVKMNSPVALAVLKKTSLAERLLAVGREERNGEFSFVPFDIRTCAENEREVWAASDEVDFTTDSEEGWVSWRDDSSEDSRQEGRVGGNRRGEEVLCVELSFPERPLQTREVYELFVKKGTSYSRYSGPLGVASAFLSSSSPAPHFAFFGAVRVSPAFIDQSVYAVVSHRHRRLKEKKGSFTGPRPFRLHGGRRALKHVSYRRLTLVLPHSLALPVARHSEANTDTLSPSPSSPSSSSSPPSSPSSSSSLSSSSTPSPPSTSSPPSTSSSSRSVARLAVEQTSATLQKAAEKLMARMQLVHVASGQALSLRATMQSKVHLVLWCSQLQPGETYKLRIVGDDAVAGESDFSPLLDGFGLALESSEIEFSMAQLRPNLDFLRCQETLWILHDRQLEHLGASHRADYGECDSGLPMAVMTVRHGKKEGEEGEGGHTATWGDVDAVALEAEPFAACIRSGDAKCVARLLPPWSHRHPPLKRQPSHELFYFDGATGVVSHESPSQLSTAVVAASSTSSSVVAPCLTDFSSNSLYLVSTHTQHYRSASISTDKHLLGALSISVFHSLHIHHDTNRLVLNFQVLSLRTAQPISGATIRLFAASVAETREATLLECDSEEPRPREKARGAWRSSGRKNACLAVQTDSNGFATWVSREILEEGIEVFATVVASIENSSPSGESATAVFVTDRLNWPWEFRHKPRLGWEAWQGGPNVLAGYDRRFFVPANEIRFFLLTDRSSFRPGEKVSLHGLLSTVNASLCGFHGACLLHHALRLDAPEKLRVLVGAQWPPETGGHYESPGVHASSEVGSSHSCTSAVVSLNRFGAFSLSLKIPADAALGSRAFLEYRIFKAGDVDEAALSETACPETWYQLRNAGNLKHIDPAGGFSIVVEDPKPPSVVVSPLKLPAVVDPASALTVSGSVQTYAGLPVQDHRVEVRFAFQPSFGETTLRKAAARLQDSWNREGKRAGQGASERTSDCGRDFSKFLIGSDQVGVNVVTTGEVSSRDTVHLHAEVRTDAGGQFELPLVLEKLTVAPSKCVGIETETALGVHPLEWEEGTEISVTVRVTGLTGDVLPPQTASVVVASSEFSLARKLSVSVRPVLPGVPFAVTAVAKPYPGVKATQLPTGSWLEVSVLRVDPQKPLGSSWEAQADNWNFWNSDQGLASCQPSLFSEAGASESAERVPNTEYRAVTEEAMEAFTDGAVDLALFVEKHEDRFSIVKKCRGHGERLSCPVTLPLDAAQYIFLTTMRVNGRRVRTCEYFLPTAGNLLTRALKPDLQLYSDVVAPGQAVSLVLPALFRPGSSIRPRIYEVRRGGGEKTGPSRQLRGALSVWWHTQSNRRLFFSVSLDSTDDELRIPIGRVPEDCPASCSVRVVLVPPLSETPLPISQVDTSSNALMPKRDYFPIETEVGARYGPFLIDETLSVMVRPAASPFVIPENVIRVSFNESGASAREPRDAELKPGKTASVRVALLTRTLEKKSALASFFSRLTSPQRQIRAYAFVGIVDKRYFDLGPVDLPQVEEEFRQRLVDQNVRQSVSSSFAEAASLATYLYLFQFLKVLKERDPWVSDLHWPQAGLLGATALTSSWAPWSKTLRNVLLGRTSTLTGSFAASPRGENLVDGVVFAQMSREATAMPMMGAGVMAQAKRSALTASRSGDAEVSVDSGETHGVAAAAKLLLSDTPLILWKSVELSEGETPGELIGEVVVRVPDDSNRYLLRTQVVVEVEESEAPALSFFRRLWTRAEALKLSRVFYGQFEKEVVAKKRVKLTPFRPKLLRKGDLARVGAILQVDETLVSEGREAVVSCWFPERNETQETGHRQRVKLTKTALPVTVQVDTDDPSLILNNRLQVNCFAQLASDASFSHGIAFAVPVVPMAPRLSLSSVWAMVSPRAFKQLSPGDGGAGGQQLEPPREDSTSVTSVEEKIELPLPVLEGVGGLSASVGVGYGAVLLGKIHSFLSAEICPFLPAKQAHEDLLWDVDGRRRTDLGSKKILCTCCLEAFPAAATPFFERRSPSLSALLLVLLARQVVKTAKLQMHGELVASARFAETKLTAYLPADPEIFRRVGFLPRPSTEYTPSALHELRVDLDVNLLVLLVAKRQASSVVLPYVASVAETIRAFLRDAEARFLALDSGPSPGDLWPQPVPLIAASEPGVDMPDSQVVAQAASRVGRADAAKKKREDFTGFLAFVGPDLLARIRYVLGSATPLNLVHPEAEEALAFPSLLAWTLSAESRDRESAKEQRLSPHLLWALVVGLEHREEANGRQLLALAHAVLKAAVGVLRFLPDSAAYFSRVAGGSVPASDAQHALLIQIASFLLSATSAERPAPSTVFSTLDPELFASGSERMSPESIVHVFSKVLLYLARGGMSGQQPLGRMVPWTGGLFRNPWEDLLVMDAVAQWHTATKSDRADLSVSVELGSEKRSTWADGDKRLMQPPWLSVLRGQLSLRRQTAVLEKKLSWTDLDASEILKPVSFVSSNFMHANDAVSDDAEQCTWHGKVRVNVHGEGVALVSIAMDFVPDRSHMLPTFMGALLQKEFLPFNSATEQCENAPVASVVRGNRVCVSLRVTVKDELRDVTIRDILPAGLELSSRDPSMSPLAVVDDAVSSVPPSSHFPTVGKRGSASFFWFLPRCEPRLLGNAVEWKCPHLAAGTHTLRVIAIATVSGFFAVPMATVEVGTDEEGGGETLSGQKQADKVMLLGASGAAKRAFVVLEEGERQLAANEVAIFKEAGLQPPPAWLLGSAPKGCGVCPAGTVCSPALGKCVS

SEQ ID NO: 59 - protein, 314 aa, T. gondii
MARVCRVAVGVRQQLAASVVAGLLVTLLTDVDASPVNALPPDPAESTVPTCDEGQEMTITLSPEKNAASFMCGTAIGNISPPLRPAKEGFEAFVDEAATTVVRFHSPDVQLIEENNVYTVTAGIFPPVGGTWYLFCLEPGIGSAAVNTVKKKCRVEVVIKGTSIIPQQCTTVGGSVDLRIRGPGYAVTFGCGLSFPQLDPPLSGKEVYVGRECSEKQQLSALVPSAALEVGPAGQLYTLFVDKLPPVGRLLCYKCVNDLTAACKALIVVPPSAEEVATTVASTSTFGPSSDATIALHSSSSYLLIAVVFLLRLM

SEQ ID NO: 60 - protein, 501 aa, T. gondii
MDTDLLVDLDRDNLLESICTEDILAGLNEDESKPDKGGNEEKLKDDSEKSAGGKVKVEDTEGDKSSRGSVDCAHLDKMTGLNKFRDLEKRREEERKQHQMELEAEKAKKPYSGKKWGITTPAGPVRPQEAAGSVVAEAVRSNKTKISAREEIEQQTRKALEKQGLLTHPVSPRPSCGEVPAVSVTSPIEQNSDDAGAASQVAVAGAASVEASGEGKHEDGAAHCSTTQSTGSQHSEHDEHEDAKDDKGAQEDGHNATDAHEVGQDDHGGQEVATGDTNANGEAGVTVVAATEVLDNAGSAEQSQVSVSGAGKKTELQKIKHKMLGLFACYNKKGVKEPIRPEESAVTVEAVTIEAVSAAGPGGNALPGSGTASTDQKEQSSGENMKCDVEQGKPEETQNAAEAEKLDSGKESPVTAGKPSQPMVDEAAKPAAEDAAKQTVEEASKQTVEEASKQTVEEASKQTVEEASKQTVEEASKQTVEEAAKQTASEVTKPTEEANTS

SEQ ID NO: 61 - protein, 189 aa, T. gondii
MLAADCFFGPDVVKRTQQGNYVPVRPDHFAGVSVALFFAKAGHSKCAQIVPVVRQFYKTTNFSGEKAVIEIIYVSLDKDEQDFERVRALMPWCSVEYKSCLRKKLIERYRVPNGELAFGTVRIPSTAIPLLIVIGPNGEEAGRMNFQQSDEFVLQRWDYRFNKWPGSAQRLRTLNDATDPWKKRLPQNV

SEQ ID NO: 62 - protein, 315 aa, T. gondii
MSGNNPSPGYSDSGCYYLCVCCRPAPPGKRIDEEELVPDSTTTEEALKEVDEESFGEEAVEDGVEIEEGETAPSSAGAEVTREAAADGPTVRTRVVTKKRAKVHPKSAVKSQPKLFTGSAAGTPPPPPEACTGPLPEPAEPTAPLGMGVYLVYATENGGTMYMKWSNTPLSGPGVLAYIEPKKEVGAFKFQKKDGVQHICGGLEKDMQSSFVADRKKYYDGWATFLKQMDAADGTLVLLPATTLQPPPKVKVAVYSQKKIRILEPDTPLEKAGVELMAVVPDTFVKFDVPTMEVSEFVAFANNVGSLISFVPAKK

SEQ ID NO: 63 - protein, 667 aa, T. gondii
MISPVASVFSTMPHWKQGARLHAPGGRFTFAARIYLFLLLSCLGFSCSGEIANGKGTDTTPARLDPRTLPRYNLKRHFPYSSIFDPAIDRDIEALSRRAREFKERFKGTLETTLLEALIKHEQLDEAVDFVDYYIALVAAVNTTNEEIRKRVNQLESAIAADVQPYRLFVNLELGAMPEAALQKQMAANGNLSFYSGFLGAARRRAPYVLSEDVERALLVRKPMTVQVATEYYFKQLGDATFDMNGEKLILSMILAFIMDNSQEKRWAAQKAVKQGLERHKITNFAALSLNVVAGSWHMERKERGYERLRSSRNVANNVSDKTIDALIHAGETVAVSLTKRYFKLKKKILKNRAGVEVFDFADRLAPLPLKSSDRLYDWKESTRIVRDAYKSFSPTMALMFDKLLEEERIDAPAVPGKRTPACYLGTPTTGPFIILEHVGQPRCVETLAHEAGHAIHSMLSYEQGNLQLAPPLTIAEMASLMGERIVFNDLLRRTTDPEERLSHLLRYLDGWTSTVTRQLMFDDFERRVHDARAQGTIPDGAFTTMWKESLEKYFGAEGEVFDSYANSEADWARIPHFHNTPFYVYAYAFSDLAVGSLYRVYKAHPEGFEQKYLDILRSGNKKSFEEIMKPFGLNPSAETFWADAVEATGGTVIDEAESLALKLGFV

SEQ ID NO: 64 - protein, 360 aa, T. gondii
MNLLVISCCFLLTLACLFEPHEQFLVAVPTRASTTLRVQPIQKASCHLRKQRTATFSHFHSDVRIVWMHSVYGSEVADSLMSGTEPAGSDYHQRDDMGQAATYFQKKNTTFISFEDLADDVRKAKYVVALTGAGVSAESGIPTFRDPSDGLWKKYDPTVYATIWGFWRYPHKIWELLLDFLRTNDPMPNAAHVALTDLQRLGYLKFIVTQNVDNLHQDSGSTNVIEYHGSLLSATCRQCGKKMRLSKSMLQDENFAKDLPPKCACGGIFKPDVILFGEGIPANAVRDANREVDKCDLLLVVGTSASVSPASDLPYRAMRGGAKVVEVNLETTGLTNRISDKFVQGRASQLAQTVKALQRR

SEQ ID NO: 65 - protein, 716 aa, T. gondii
MMTPECGDSPAWSHSISGNASINGDPSCVDAATGEDPTELRCYYIDVAFDCVSEVNTTSTETKMLSKLWGDESFSVSEADGRADLPAPKQKPSSEIVSLKRQERVSRVARRLYVHLPRLVRSPMTRLQKKTEKRVVASLPSLARSESVVTADSTGEASCRRLSSVGGALSASGSSLKRSCSRGRSQAGGKVCSCESIFGVFTLRVFLAACILMLALLIQLVLLVLARNLPFAHHSKGSEVAAVVSEQVTAKVGEFAQLSRAAQPHELSGEDTAVSSSFITLPESGFRDVERDGLGTTSRFHRAEPAPRSVFACNVAFLIFLFCSVLRMYFLTPNLASAVTIRFFLCVSVAFLFRGLSCLLSALSNHSAVENRETQKDFFPHIVLEATGLWIFGGEAGSPVTSQKLVLWILVSFWGYYTSKHVFLAYIVIPLVAVIVCVIPTTAACDLPGHAAATLFISSVCIIYHLLLDIAAQRYLRTQSFRPSGGSIAAFCGRYVVGDVLIRVLAFLEALHLRLEGVMCVSSPTVVAHVKLPDRAEEESVSTPHSTPHSLTYEDLASRVVLAYAGSGDFDATNCRRAFLCLLKKVKAIGEQERCRESGGEIPTAAECEMEVFAASHAYRSNVNASLELGESGLYLSTSVRLGCAFRLARVFLRTGICFTPMAASPREETFYDDGLSGMPLLPRRTFLVENRRREDVCVPVCRFVTRMQVSRISKL

SEQ ID NO: 66 - protein, 347 aa, T. gondii
MLFPPGIFSEATAFSHKRSIRSISSHSTFDDVTAETDEAPVLAEVEKMPAVVKKVKHGMRKVLESLGILDSKCEQKKKHNKIPSAAAGDSPIKTFGYPFYDTSLGRSLLRPQVGLSFIEGFMQPIKVGAFDWMVQGTVDDVLSFLVCFDDYEAIAEKLGEDGAWHSEGNIGPLYLQLQNTSQYQGDASSILMAYSVEQILGRIDTWGVIDQTIGHWWKPAASLSEKAKSVYDTYQSLKERVPDLTTEKFQEVWNSASTKSGVGKLKELAKLFTLNPETRDLRDSWENLDRVDRGRKISLYVTSYPKRSRTMATFAFGENRVKLGDMAAAVAAATKDSTLDNLLKKYV

SEQ ID NO: 67 - protein, 168 aa, T. gondii
MEKMSVSLKALCLAPFNASDFKAAVFGGLFGGLASFLVTHLLLELTFSPFFSVFFAILLASIAGLVIQRALAIDPPVPPPALGFADEDDSLDLDPDTSLHSLLAARLGRGPAPDAAPLSDNAWTGRTGSSGPGGRGNAADAKQMSTEEFLNDDEEEGAMLFGHNALVA

SEQ ID NO: 68 - protein, 337 aa, T. gondii
MIPPLLLNSLLSRKAIILQHSLPCKKKRRLAAVDSDPVLLALCSCARILVHSSPVCAAETRMTATLDKKIAFIGAGVMAFALAKGFVDSERVKKEQVYMLVRNETKRSLVEDLGYKSFQNIAGLADVDIVVISVKPQDAVQVLCDIRMVVDKEKHLLISICAGLSLDTLARALDPSALNRRICRVMPNTPSQVARGVSVFALGEGCTDEDRVTVESLMTAVGSCYRVQEKHIAAAGAISGSGPAFIFTLLEALSDAGVKNGLPRKLAQDLALDMVEGSAALARVEFGRRHFAELKDQVTSPGGTTIAGIAALERWGFRNAIIQAIDATTDRAKDLDC

SEQ ID NO: 69 - protein, 2473 aa, T. gondii
MNRAVCTAAGVTRLPSVTAFPDFRLRLPLRVRSVRFIVFAVVTVFTFSVDPERSFWRVQNDRLVTHFLGHGHSSEKTLFALSPVLAHAITRETPRKTLEERHHVRAFSSQHAGRARHDEAELQPVSSKDSTARRTAAAHEESKAHNREGKGASEGFQGRSKVENDGQESPDSKNSGAPSAPSSQAKPERNYQTGFLGFFSGQCPATPLTTPIPPHFVRFVIICYSVIAGIAILWLLVQASRRKHHQRKQKQALQELVRHGELWHRSGKVVQRLSSGMRVATEGDPDEDNSLHSGPLTFVRGMLIQQEGCYRSLPGSMIKTVLKASFALACVLPILAISVSVVTHSNRSLTSFLMPPVFYDAQEPPAPPSNFRLGSESVKSSPSDSSRAIPKTRPPASLEGSSNDFITQYWISDVECMQTREEVCVSLMLFSFLYLALGQALWVRFLRDLDLTPAPLASCSQLRLRVTYIPLHRVEQLRRSWQREHRCHAAKTCSDELMRRRFTAVAASVTNVLSAEGAENSSQALERLGAGEACTSAVGHPGKATREGSEEGLEGKKDWTDGGMFVEEEDLTRWSMGEINLQSLQTQTFVADVWSTVSVQHRQRFVEVEGLSFVYESRTGVFVLATTFQEKQGVGEAVDLAEALTAEDMDGSEDKATRLLNTFQRVLLKPEEVADRQYIGKNRLVVANTTFRELVWSSVTGNAFYFAVLVAMWYYSFTRNFLVLGTLLVFVVFEGLYRIRLLVRQQKRLQSLAAEREKAVSAKPALVLRLLRTASGLKTGAEPRSATPPQSGQGSHSFVPTWIRIPAADIVPSDIVRLSRGDVVPCDMLLVNGTVAVDESSLRGDGTPQRKGPLRVSVRKLRGKLHGGDKGTPLPEDGRLADSVLHAGTSVISCTEARGRSRTLDEEAIQYVFTVEDETANRSAGKAFRETLGVEQRAKLEKNLATVERTQVAAAEALMDAGASGQGGICWGVALRTGIDTAAGQQLRQLQLPEQEMFRYDRKLIYVCSIVLILWLGLVAVHAHYTESLLLSFRFAVDSLLKLLPLWLPALCGLFATLAARRLRVCSAKEIDGFRRRVEQATGRNCLRVFLSAASQARMLASLPSEQPVDTREPQGMSPVSPKSRSGLSSPLDPADRSSTVVDSRPFTVVCPAPGRLPIAAKVRIVCFDKTGTLTREEFSFVGCQPVEAASMLSFVSYEPDGPAMQMRPRGAGAPLPNVKNSPQTFQAAGGDRQVPPRLFEGLVCCHGLTLDNAQMVGTLLEQQMFESTGWKMKWTVFPQQRADGPTEIAGLTRLAFSPANAKGYYSDEDGDRTGGFVLLQRLVFDPVRQVMSVVVAKVKDERRGDQNEGEVFVFCKGSYEAIASLCRPETVPGQFLHRAGTYAKEGVYVLAAASKSLGVRTDLNAWKDLPRSEVESDLDLEGLLLFRNELRPDAADTIHQLKVAKIRPVILTGDSPLTAVAVARRAGMVGGSGGVFGSDTGRLQRLSRGDTVDGLHPMVLGDLVDDDLSGEDVEAFQSGQDRVGDSRAGKRCTGGSQGWHPAKERTSAVCQGEKSKAAAGLCERVKWTNVDTGEEIDRWTVFFTKEYKELALTARAVEALTETPDILMAGDLSGEDFAVGDEGDSDQLEEESEGLLWSQGHSGVPPGSESTPSNTGGSSGSQSPSSASLGQTECWSPNSKRYGGPVEDPSSLFRVRQRRPTMFDRILFRVRVFARMSPHGKALIIERYQERGLIVSMVGDGTNDCFAIRQAQVGIAFGPGSLCQSIAPFAILTNQREEPTHSASSSDSSASAGQSKASLVVHHCPRANRFDSCGLLGVITLMREGRATLVTSFAVYKLQILYGLLSAVSYLMLTVGAYGTPNAFSLFFSSVAMLLGLSLSMLWSVPSVTPLTKRSPTSNPLGVRTVAEVMSILIVDLLALFLLFGLLYGPAGRPLPCAWVQREVRHELLQRQQIENLLDLHSFNEPHIAQMEDAVTHAKKKLVEYNPDKEADGGHTKQRTAVHDKAIAEVQRWRVEVTPSLSFPTHEANRVTDLVGNVSDKTISSQQQTLNGNHSTAMLKNLEETTKGHNGATAFLEVNQQVATRFRTEVNAVPFREKSIRKQSVFSSGLVEDVELRNMIPAAKRNRAVSHNGNAHEDGEVRHFSIPESSAQSWIEKTRGTAPPPHPDVDTLMGHNLRPGAAEHNLPCSRDGRTEASVIFLWLGACLLNAALIFSSGRTSGKAFWSNPVLMPLSFIFAVFFVFLVTAPKNRVSCVFMVNCPANEIRMQQQRRNAIGVAKQLVTDEEAKDMYRLLARNAEMDVVKVRAILSVDMAAPNERLPTLPSTSLPAHSNLGGASETSKSGQLETAGDLAKSFRARMARRAQIGIHGSRKPMIPGQFNGATEERNEGVNNVQVDEVQPKQGDRGRVKGNNGSVISAWYGQVLLYVLCSMSVLNGMIHMYVIGDQMGRDTIANWWRKAHPSRYKGEVIAV

SEQ ID NO: 70 - protein, 719 aa, T. gondii
MRWSGGPATASRPQTTLSTQSVPEMVTGFLVFWLNGPTSKEEHLFVYCGADVGKFSLLPRPLVSECFHVHWPGARASPRDVRHPGAATSAFLKALEQQILSDFRRRGLWNPNKEDGTKPFEFEIDLYERGSHYGGRLDYAVVDGNVVETGGADIEESNLWLSTFHKMLNNHISENGNKAAADEDVGSTGDAAGPMPLAEFESSVTRTFLITRDGGVRDVSIPAFFLALRGNGQGILELMQDTQKGWKSLYSKLAGIPLCVYVTRDLFLQPDFEHGSGEKYEELCAAPKGFTSGLEMVDSVGMKPLTEKTFATQAAETGLTPDGMDFMSGVTRSIYSQDIEEINAAAGVVAMLGSFGSFFQGKRYSGRVLVEYLIARFTSNAFLNCGIRDVLEEPQSGARQVTKSRKRYRLRPRLEGDSCTAEAQRRLESILYDFVVVAAPLELSGVRLYRHREDSWKEGERTRSEASALERVTVPPRSWRTVHLVYFVADAIRWTNSRSVSSEEGSRSGDMSHLILKARPSGASAGAFPEFYVAGCYGHAVEDAGQDVFRRKVSSDKTAMGLDLGENPRDYTATPESDDVAPGKKTLCRVASPQWLTDETLESTFVNPQHIYRRRWLAAYPNPAPFDPVSTSATAEQFSSSASSAQAFNLNASPSEHASRKRTTTQHAVPEQSNFILADNVFYPSAFESIFSCMEGQAVSAQNAVNLISNSLDIYSGEV

SEQ ID NO: 71 - protein, 318 aa, T. gondii
MRSLKSIVVPLSAALVAAAELDLFLGESGVYLFGKASESDVALKVPEDPVPEEPRREPEKHVDLFGEDWKQFGGSGFGDFSKVEFENLFSQVHEMMRRLMGRGVDGFGPSLLGDSPGFHFPRLRALQPKTKLEKTGTCQYVVTWAPEVTAENVRVILHLQRRQVEVQYRAATRRDEKTEGGESHSMSKEQSSQLMSVDPQCIMTREVVAQKLAGWTDNTHTATAGTPKKLLISFPSPDHIKEMVKEGYLPDNALERVLAGDFEGFSRTQMCLVSGRNRTECAFAEGQEVELEEKPLPSDSSPVTSVELPRLSQEDRGL

SEQ ID NO: 72 - protein, 377 aa, T. gondii
MANTSVRRRQLLSSVLLLQWLTTVLGVAWGPNPIDGSKHGQFPSLRRTEGVSQSGSGHRGSVYRIPLADMTFWSWMSYLKELPDIDESRNPILKRLLSGSFLRRDGSTTVNVRVPARELVRLLSLTPEQQREGVSAKVRLINLLDPKYSVYEPYLYREILPKRSPLLLPSLGEYRGAFLTYIFHPLSKGLVGDMLETGRSHPDVQVLAANMVAALKSLHNLGLLHRSIELNSFSVLPDGTVVLGGLDTAAPIGTETRLWVGFFGQETAPEIDRNFLADLALTQGRHTVKSDVYSLGVAFRNLVQLLGNGNLGPEDRGAVRQDHLELLDKLSQKMIEEEPGNRPTIEEIMKDPLFEGLNFEDIEEGKARPFRYKQNRL

SEQ ID NO: 73 - protein, 248 aa, T. gondii
MNVFEQYNQRQGAMNLKHIFNFAPLSPIQQEHLTRVYGALMTNIILTAVGVYVQQRILALPIFLLLGVQVFCVWGLGASSTEAVYSGKVTTPLRAAYFGGFGFTTGMMLGDYLYFVNVLNPRIIPTAFLVSMGIFASLSAAAIVAKDRKFIFLGSILGTGLTLFTYVSLFSVVWRTKLADDVLLWGGLLLYIGFVLFDTQVTLEMARRGSSDYLVQAIQFYVDLVGIFIRVVQILADKERRKRQRDEE

SEQ ID NO: 74 - protein, 229 aa, T. gondii
MAPSASHPPGACPPGCTKHPATATAISPSGVCPMRAFHPAGPHSHFSCYDDLRNRLSHDKNVRPVASQQLDYLDEVSPFALAYYPPPFWGGVGLNPIDDMLFETALTANEMMEDITWRPRVDVEFDSKKKEMIILADLPGLQKDDVTIEVDNGAIVIKGEKTSKEAEKVDDGKTKNILTERVSGYFARRFQLPSNYKPDGISAAMDNGVLRVTIKVEDSGGAKQQISVK

SEQ ID NO: 75 - protein, 468 aa, T. gondii
MVGVFQLCLLTCLLCLLKGSDAIQLRQHRNGLGVEQSFVSEETDIVGGRISSLQAELDSYCHNRYKQLCDGGNKKFCDKTGVARYGTGIQSQQTAEWRCYFAEVLKPSGRKVQCVDDCGNYFPCLGVVDPNDTFHATAHNQILNFIKDGVEKHCSPFQMAGNNYCQGVLADTVARKDTGTASQKAKAWRCYKKDSLTYEARSICVDNCGGEIECPGGRSETSGELLSQHYTREKELQKVIESQSAPCHDACVATPINPPICADTESLLQSTKRSRAQRFIDDACQKLFNCHCKKDKKFCTTVVARKDRGRAGSQNDAEWRCYSLEELDFQKTNPSCIDECGNELPCQGAVPEESTHHITWTKLPSKIDEATQKFCTERQRAANDYCASEFADSLARYGPGAGDQTSQFRCIKKAAMRADAEGQCADSCKGTETCGGGRSRLDGPLSVDDVLNAHEGISEAMKSASTEC

SEQ ID NO: 76 - protein, 224 aa, T. gondii
MATTHLNKSVIAGGSIKTIKALKKYWNSPVSDIDDNSSEAKYTMLQMAILLNKKNVVEYLISQKDVDLTTRATDGTTALMTAVGKNVPVDWIRAMLERGAADNINVEDNEGHTALDRCEKDSEVYKLLVQHGAQPRPSPPPTPPPEPDVAGGAGSTDTNAAGQNGASKPVDGITGVGGMSPGLDEHPGIWATMCGCGGRQGKNGTEVVEVVDAGKAELNPAQAS

SEQ ID NO: 77 - protein, 866 aa, T. gondii
MEDSAVRYSSNVPLQETPAWGGGSEERHRQGSPHSPCAPWCRVRCRLSVFAWHFLSTPSFSFLRKVFCCFRNPPESSESSAPRNAATSGTEEHGTLVADSIPPRPDTAPAAPWDVCTPRGVAWKQSGRQSCLFAALSASFLGSFLACVVLYLLCVWRNDWQSIDTTLFAWSGKYWSWAWILCSLFFFVWSYNVVLSVSILLVLRPPPCWTRAAESSTSFPAAMSSSASRLSSACLPVLSPLHYILLPGSLALCAAFFVITFLLWGPEYRGVPLWFEFYFPSLYAVSLPVVTLCFGGVIVFFSPTRSSSPSRGVVFPESSQQRPGCHPHSSAPLLDTAGPAAFPGPPGSAYQPYSHSDLCLFDGQECVFTKTGTARRASAGEADLTAPLTGSGSRDVCSPDSPSAAARGRASGTHSGCLGVSATEEKSEDRAGDGGDREACSEEDSETEGPVTAVHQWRHVVFCLPQWVALLVLAGVWTFFLAAPFVAPWLFSSPCLLRDPPASSPENERRRVKFSGEEETWKTKSFFAFGSDSSSSLNTHRSKRANLHPWLPEKPLLIGHRGLPELRPENTEVSFEAASAMGCSGLESDVVISADGVPFLLHDLTFARTTNVADVFPSRAKTRADLFTWADVAELNAGRWWLEKDPYGTVKLVDPVVQKEISEQKIPTLEWLMRKAVSANRTLIYDLRCPDCDSNTWGCGTKCVDLTIDLVRKTKCSRHLWWLQDKRQEVKKEFPDVTIVTAADRHFRHDADNLTDVLNVEWVQLDAQLIKMWNERGYWVNAYVVSQPWLLSYFWCAGVDSVTTNSCSRLNAMDAPVQHISWNAFLWYVAILDLICILLFIGLLYFCRRPPSDCPCSVTVVNMSSF

SEQ ID NO: 78 - protein, 252 aa, T. gondii
MMIRISGHVCGGGRPGIPRWKSVLRKYIASFCFFVACKTWPGFVSCSIWRPQGTPEVGSLGHDAADTAAAEAARDVLSAWLQEVKSLIETAAYGVRGVANDVVDGHIVEEALGMTYDIHDQLQKRIAEEAKASEVRIAQAREKASQILERLQKLDLSSISSSIQQVPARELRELLSLLAVPRMPSLSLPQISISFNKDPNSETDENNQDKGAEEAQRPKQTASDATAEDVEAEIDKSQVPPSDDIVQSTSDV

SEQ ID NO: 79 - protein, 444 aa, T. gondii
MVVIKDIVAREILDSRGNPTIEVDVSTEGGVFRAAVPSGASTGIYEALELRDKDPKRYLGKGVLNAVEIVRQEIKPALLGKDPCDQKGIDMLMVEQLDGTKNEWGYSKSKLGANAILGVSIACCRAGAASKGLPLYKYIATLAGKTIDKMVMPVPFFNVINGGEHAGNGLALQEFLIAPVGAPNIREAIRYGSETYHHLKNVIKNKYGLDATNVGDEGGFAPNVATAEEALNLLVEAIKAAGYEGKIKIAFDAAASEFYKQDEKKYDLDYKCKTKNASKHLTGEKLKEVYEGWLKKYPIISVEDPFDQDDFASFSAFTKDVGEKTQVIGDDILVTNILRIEKALKDKACNCLLLKVNQIGSVTEAIEACLLAQKSGWGVQVSHRSGETEDSFIADLVVGLRCGQIKSGSPCRSERLCKYNQLMRIEESLGADCVYAGESFRHPK

SEQ ID NO: 80 - protein, 452 aa, T. gondii
MDCGQCRRQLHAAGVLGLFVTLATATVGLSQRVPELPEVESFDEVGTGARRSGSIATLLPQDAVLYENSEDVAVPSDSASTPSYFHVESPSASVEAATGAVGEVVPDCEEQQEQGDTTLSDHDFHSGGTEQEGLPETEVAHQHETEEQYGTEGMPPPVLPPAPVVHPRFIAVPGPSVPVPFFSLPDIHPDQVVYILRVQGSGDFDISFEVGRAVKQLEAIKKAYREATGKLEADELESERGPAVSPRRRLVDLIKDNQRRLRAALQKIKIQKKLEEIDDLLQLTRALKAMDARLRACQDMAPIEEALCHKTKAFGEMVSQKAKEIREKAASLSSLLGVDAVEKQLRRVEPEHEDNTRVEARVEELQKALEKAASEAKQLVGTAAGEIEEGVKADTQAVQDSSKDVLTKSQLALVEAFKAIQRALLEAKTKELVEPTSKEAEEARQILAEQAA

SEQ ID NO: 81 - protein, 238 aa, T. gondii
MKVLFFLGLLAGGLLCSADTPSLDSDPSASPLRAVLHLRGPSPVPAQVEPHEADGSYLEATTGNEHENTLSDESEQEEADIEEERAAVSALQMTQKEAPNTGATGVAGPEQCSCEFAGSCLPKGSCLGIAFTLVAATLFFVIFLAWLLQWIIAIPSEWILAKRLSKRDTSTKNSPREEDDGRQALLQENDSLDGRQDEAKATTEGTAISREEEEERERTIRVGPSGLPPPSPKESGRL

SEQ ID NO: 82 - protein, 499 aa, T. gondii
MKAVALRGFWLTILLGVFIPRTASKSSGLTSAAPDFTVTIPKEGLPADRQEVFSLRPSGILRVIDETGEAVYMPQATADSDSSSVDPSKETLKASDAVSTQTYGDAYAFVNGKCDFRETIKYKDTFAGYTAPLWVRVTSDASMTPETSSSAVVNYTFTNPPKEYLSEVVSFCVIFKTRLASGSTSSSPAVTKPTEPSGAAPQSTSATLSVPAAEQNTSQHYGDSGTGHESVPEGKPDLGKDDKVNKEIHGPKGGPGPTGPVVPLQKEPGQSPDTPGPLTPHDGTASPKRKTEEDNGKSGVAPKQPVPVKPAATKPSTTRHPYASESPSDRAAHPADDDRGYSISGSKYHKQGGDEKSVRDSEVAATGPGEHLHVEQDRRKGDDVAHNAEEEAASEAASKGGSMVNDEVQGGKLGNDDHPESAETSLQGGHRNILQEEHVDSKDPAEIEKAHTRRLSDTVTPESAHLTIVIHSAAWGLAGGRAAIPAFVLSCAAALFSTL

SEQ ID NO: 83 - protein, 172 aa, T. gondii
MTKNKILLRAVLCFLILFGCSAWRVRAKSWTYDFKKALDDDETKKEIITPGDSVSIENSGSRPLEYIPPNPSQVLKVEKGDHCKDEPVELAALFKGSAPTPAWTEAQSTRSLTVPAGSVPEKETIPFCFKVKDTGKNKTLTAVIKVAGAHGLSAAVGVSIGIPALAFVLISM

SEQ ID NO: 84 - protein, 365 aa, T. gondii
MSCSCPSLCEIGDFRFPAGASSLAGRLPCLTSPRQRSFPEHKMVSHTAGCSLPWRRRLGVFSLVATVQGALYPSAVLSLRMSVGTDTRDSSLSPPVAVPPSAAAASSASSWFNSSPSELSAPSSSAPEPPFFSPSALGFGQLAPPLVMKVPQMPASSLPPVPDNSETHEPCLLPSPISTQSASLSLLEEAADHTVPPQESTASTESAASGEAVSSPPSDLSCTVAFEGPISRAPTLTLSSSSDAGPFLAIFRDTHPSANGWIHGFHKELRTGYKGPFGGENGEYVRCHPPAGAHDYEVLVFDQDYELGPKLKAMAHTTWNTRARALGTEEDLIKDIAHNAPSGATPKIVTRCSVTVSHEQIAEGQ

SEQ ID NO: 85 - protein, 577 aa, T. gondii
MFGSVFVLDSDPMGFIGNRNVEWTTNLDFFYCAFFSASLLGVLLAFFTDDVSSGSLRWSWIVMELLPVPRLSNHVAVKDVEGALITAAKQASGKSQVFAKIVTAAHEGTLKVLLAQWCTKLHLRCWFCWHTLKLRYTAESRRQLLYQVNKVLLRLENRKGEKEVQSYLDIKRYMQTNNLWYFAFRISDVKSQYITCEGKRAYHMSSYSYLDFMREPLVQEAALAAGRMWSTGNHGARMLGGNPTVIRELEQIIGRFFGREDALLCATGFLAAMSSICAVAKKGDLIIGDNRLHTSLRVGMKLSGAKEVLFRHNNWQHLTQILGSMRRKYIDCWIVIESVYSMDGDIADLPTVRRLADQYKCQIIVDEAHGLGVLGKSGRGLEEHFNMPGAADIIVGTFSKSIGGVGGFITCGKDLIEFLEYHALGSVFSAPLTAYSAGGAKKAFELMQGEHRWRIAKAQENAIYLRRALKTGNGNWPPDYPADKKYEVEGIECTTVIPVVFPNDPYRLCCVTRALFSKGWVVGAAMYPACPLMRPRIRITATAAYTKEIMDKFVRDLVKTTVDVPLTTEVEDGPITL

SEQ ID NO: 86 - protein, 326 aa, T. gondii
MTGTVSRRKKIAMIGSGMIGGTMGYLCVLRELADVVLFDVVTGMPEGKALDDSQATSIADTNVSVTSANQYEKIAGSDVVIITAGLTKVPGKSDKEWSRNDLLPFNAKIIREVAQGVKKYCPLAFVIVVTNPLDCMVKCFHEASGLPKNMVCGMANVLDSARFRRFIADQLEISPRDIQATVIGTHGDHMLPLARYVTVNGFPLREFIKKGKMTEAKLAEIVERTKKAGGEIVRLLGQGSAYYAPALSAITMAQAFLKDEKRVLPCSVYCQGEYGLHDMFIGLPAVIGGGGIEQVIELELTHEEQECFRKSVDDVVELNKSLAALG

SEQ ID NO: 87 - protein, 165 aa, T. gondii
MSDWDPVVKEWLVDTGYCCAGGIANVSAEDGVVFAAAADDDDGWSKLYKDDHEEDTIGEDGNACGKVSINEASTIKAAVDDGSAPNGVWIGGQKYKVVRPEKGFEYNDCTFDITMCARSKGGAHLIKTPNGSIVIALYDEEKEQDKGNSRTSALAFAEYLHQSGY

SEQ ID NO: 88 - protein, 982 aa, T. gondii
MTEDRASDPGWETVAFQAPSRLPRKPQRTSARPMFHCLLRVTFLFALSFLCLTASEGTMPAYENTLQRAQINDGQSHARHGSERLTEESAAYVQREALHEEGAAEQATVEGNQERKPDSRTRRDVDGKIPCLTQAWSATGEQKEDSCTNLLKAAEAGVRRSASSVLAEGSEERSNLGFLQWNEGGGARPYSWRVAQTAGRDDSVPVGEKLMRRDREQVGSINHHGHQEGNREGKAGDQVLESGTMDLFDEEDDPNPSLYLSDGDEPAALADPEDEDFIWGDEDEDGPFLDGDADEYSLSYDVDAAEDALNLRENEDPPNEGGMNVDQEADEPFGVDAEADTETANAAHTRPPDHFLQRYNDDVVPSPRATPLPADAEEPFVSASTAEVNGLAERKEFAKWSQDTAPLVVPNKHEEGDGIGYQGLVNISENESSSPARTPRGKANIPKPPMGWSSWNRFECDLSELNEKLVMDTALALEQSGLHAAGYEYVMLDDCWSIKKDEERGAREPIVWDAKRFPNGMPALASFLHSRGFRFGLYTDSGSRTCMGYIGSADHEEQDAMAFQSWGVDFLKIDGCYAEPSEMGMLYSRWSPAFEYAAAANPDHKQTVVLSCSWPAYVHNPTDFDFKLIGEMCDTWRIFDDIQPTWESLSAIMKFWGDNQGIFANVVAPGRFNDPDMLEVGNGNFSTAEGRTQMSVWSIVAAPLILGNDVRNMTPQTLQILANPEVIAVNQDDLILEGLRVFESPNTMSIWMRPLAAGSTAVAFVNLSSKPRNVTINLSELQKAYWESWLPWRRRKLLRLLDNIPPADRERLVQVHFPPVDNDPTAPFGCTVRDVWLGLNLGFKERYIVSPYILAPHDTFMVIISGCTLTGEPHRFSSANDETQSPELRKAGVRERDENTGVRRENNNGEARGTEPDIDILSGHVSVAGHVEQVRGITGSGEQQRNSPRQAVGEEAETYPAVVANQGNIPAHSLRSRIDREM

SEQ ID NO: 89 - protein, 190 aa, T. gondii
MGNMCAICFNPGKAASCSCFNLAVAVLLFAVYYGLVGGMDLYQATKSHPVLVTQKYNAIFTLSVATALLVSVVLGVLKLGIVSYIFTMMVFVLQLSDAIFKLVTFILNWVDWGIALHDGTMSFQSAMVTSSISQVLTIILTFSMANILYSAAMVYKVGGNGCEYRNYKQIESSKNASSTKKEDNEAATEV

SEQ ID NO: 90 - protein, 913 aa, T. gondii
MANAADENVFANDSSYHWEMRRKASFSKLTGAVPRAIPGMYNEEDPHADEKKEKLWKLMETYISSDIHSIQRSIVNHVEYTCARTRFNCDPESCYRASAFSVRDRLIETLNDTNAYFHEKDCKRAYYLSLEFLLGRAFQNALVNLDIENNYKKALAELGFNLEQLYEFEHDPALGNGGLGRLAACFLDSMATVNLPCWGYGIRYTYGIFEQKIVNGRQVEHPDYWLTMSNPWEIERPDCTYAVRFYGSVKEYRDVQTGRMRSKWVEGEIVQAMAYDNPIPGFDTYNTINLRLWKAAPGKEFDFHLFNVGRYLESVRERQRAESISAVLYPNDNTLEGKELRLKQQYFFVCATVQDVLRRFKKVSNRDWNDLPSKVQMQLNDTHPTIAIPELMRILLDVEGLEWEQAWDLTKQIFNYTNHTVLPEALEKWSAELIGKLLPRHLLIINEINFRFLNEVRGVFGDDWNKISRMSIYEEGEEKRIRMANLAVIGSRHVNGVAAIHSELVKKDLFPEFVEFYSRQGFNNKFLNVTNGVTPRRWIYCANRGLADLFSNWLGSDSWLKELDMVAGLQNHIDDPQLRKEWRAVKRENKKRLAAWVEQRCNVKLDVDRMLFDIQVKRIHEYKRQLLNCLYTLHRYLTLKKMSPHERENVVPRATMIGGKAAPGYFTAKNIIKLVNNIAQVVNNDPDVNQYLKVVFLPNYNVSHAQVIIPASDLSQHISTAGTEASGTSNMKFVMNGGLILGTLDGANIEIREECGDDTMFIFGAREHEVAKIREQARNGNYPIDGRLREVFDFIRSGKLACGDGQAQSDFVAIVDQLCNNGYGHNGDFYLLIHDFQDYCRAQHVVDETYKDVEQWTTLSIKAASSMGKFSTDRCMREYATEVWDIEPCERPPPDEFQRMRSFANDIPNKVSA

SEQ ID NO: 91 - protein, 195 aa, T. gondii
MASPTSASSKAPGTESEACGHRHPGHVGATHTYNWDEFRQFLDSQGSLWHSAVLGAPASAAPNTIFELAPTAAEAGRAIAFRPRLDAYYDTAAHKIVMLFDLPGFEKKDISVEVTDHAIIISGTRDRLNDKVLYGEKSRELIKERAFGHFCRKFQLPTNAVEDAVTAAMTGGVLEVTVETREEEASHTKKKIQIA

SEQ ID NO: 92 - protein, 368 aa, T. gondii
MDIQAVGSVLASALASPLLLAVACCASLKLAAGALNFIWSLCAAYLLRQADFWTMLLPEKTGYWRNRVAWVTGSSSGVGLSLCRLLAHRGCRVIMSSRKIEDLQAAKQDVVTFCSLKGVQKSENDFLLLPFDLLQLESFEDIVVKATAWAPNGRIDFLFNNAGIASRGLFMSYEAAEKIIKTDLLAQMKLTKLLLPIMSKAGFGHIIFTNSGRSKLVACGHEPYSVSKVGLLCFAEALSRDLKAKNMNIFVTSALPSYIRTKISYKTLGPDGTPLTDDTSYMHTDTAAGLPPDTVARYMLKAASNKLRECWIATTPVLFYLYLQAYLPDLASSLLDLRAEAHALEIEQEAQELEEIAQRVSRCPPHST

SEQ ID NO: 93 - protein, 398 aa, T. gondii
MERTGNMQQRLGGFKSQVRKLMAVCIGGILLLSSGQGLADSLHEGLQSLSLKSQVGVSSKVDVTGTHAKCEFSTAGAGSSTAVSKQSLTLSKGSLTATLECTAKDGGTISSIPNPLAGNVCVTKQKQSETPCNFGENGGAAASVQVPLKDVLGTTSAVQWMNTTAEQKAIQSQKWTLKLNEEDLPISDKTFDVGCTYTTTGKAAANPAVCQLTVNVKARASSVADENVVTCSYGAESNSEALKVDMTTTRNTVTIDCGSEGTLNPAADSAQYCNPQNKDLDDCKKKFVDILPNFVISWWKTPTPGNASILTIPAADFPESEQQFRLGCVPNKAPQSDSQDTRVDNQSQVQSRTSAPTTCSVLVTVKAASSASYASPSLQTLIAVSGAAVVSGFVVASL

SEQ ID NO: 94 - protein, 420 aa, T. gondii
MVRTSLIEHRTGRRVVAAPDRGSLQVCIVFNIALSATIAAMMTSPLSVASMTSPLLTWDGNKVTCHPEKGDVDDWIGLVPQQNEVTFACEGKGVTPVPKNLVNSKSREVCAQGMSANACEKDPRPLSEILKGAQNDWLNGEDLSRGITFRVPKNNFPGLPRIFRIGCRTRSNICMISLHIYAKSAYTSGQVTECAYESNVSLPPVRITPATNHATIVCGPYGGISPLDYKKEFCTGEPHTSCGRQKYADVLPRYTDAWWNGDPSTAEGATLTVPNGHFPKETQTLKFMCLERLDTQPRRCVVTVEIAAGVSGSKPSGGESIPPQAPGTEGSRKEAPNTNNSGGTPTGGGSDDDTTAPGTGSSGTDSRGDLGDGRDQDAKGGMSRGNSESGSNGGATQPSRLLGLPSAVIGTLAAAMFGAV

SEQ ID NO: 95 - protein, 916 aa, T. gondii
MRRYTAFNTRLIELSASRRATSYSVLFPSADRFTMSFTPFFVTLGCDADEYLIIEQLVCCDHSDLTDAPSCCIVACVPCPPRCTWTIPSDESVLRCCFLATPICIVMRFVLSLFMMECAVGRSGIPTKCRCFLGCPFPATSRSSTASRHYLLLFFLDVLVISVTVDIYVRAYPIERVRAHTGDERPFNVTTGSSERRGNTPHDGITWIAEHLADTDSGKDSHDYRFLNDDQHNHVEEGDGEVGGRTAAADEEEESSRILPTFTVQDIPSGDADVHKAAGDVDTSTTTTAVDEDAVGMPTEGDIPKGDKQVYEAFGRQGSRTVVAEVVEDDSKDSRASQETMDNINHTTQRLLRGMDDGAFVRGGGVQEFVKAMTVPRIEEKTKGQLAGVLRLIEALEAMKGSNSKSDQSPRRFGCSVLQRPFRTVVDYDVVITTAAALANAGVNVAAGGGGPVFPVFPDVAKVRSLAEEPLDGQQAAARESQLRSRGFVVPVADMVAAVKREWSEEPIDCGRCTVGGGYLPVRLLKKEVDEGEELLHFADVEYPTSISRGTVVSVPASWLIVKGLSLRELTPGVTGFILCVENGEKPVFVPRGQGLFSQYAEYRAGAFRERVAVDQFVIVRGSRRNESVLEAKLILDPRAYSVYQSVNRYDPSFLFFGTIEGPPITQSLFVTSALKTSNECIIERTVDDGPVSLDCKGWRKFERRMREYEETKAAITKRSRWRLIKYLVLALGVASAGLLYAGHRKERPHGILRVRPSQIMKHKYYDKIMVALRGRRHAARGYWKAFLDRGIQELLVPQPALHLLSYFDAMHPENLRDALRTVRGDTDTVSRWMDWASGRREAAKGVLYKGAGGYGMAATGVIATLYGLLRSGTYAYRRSKLYLRGRKVKQYAANVLSQKNGRRKARRMIVFLVVQ

SEQ ID NO: 96 - protein, 2451 aa, T. gondii
MTAPFLRVYTDILSERKVRVEGTWHLVSIKATHDQPLCACKQTWSVHFAWPVDTMKLSYFFFALSSSGATLLLFAVTQLATQVSGFDLEEPRDLRHEMKKIEVIHGSEGARFECPVESVLLPEQAMSGDIRAATVFAVAADGSCNIFDPPSLLGDVVPGAYLQEELSVNADKAAKTYTLVIPGLPAKEVKLCYVCAHPDNPAGSQVTVITVRRSGDSENGNPASSPVCRPSFSLEAWALGVRQPSVVLDVAAPGQSVRFSCLSTATELPSEAGARPAPAQVYPVNGRGWCDLSKGPSSLEKFLLGAAMTAEVRQRGGGFLTTYTLNVPRLPSTNRRFCYVCPRNRDPADGCAVLVKVRGGMVEDPIGKPAAVPTCHPQESPEGIAAGTKSAALILDIVRPYSSVKFACPNNSEVLPHNAVSDDGLKASVFAVRKDGSCIIGEHTLKLQDVVPGATLTGTTLVDKGSVTRVYTFFVGMLPTRSQKVCYVCARNSLAPQGCGVVISVKGKENGKPAKVSVCEPQYLQGVAERGLLSPSVELLVDKPEGVAQFVCPGNSVVFPEHATDESPGIATVYQASNANACDVWENPVKLDNVLQGATLRADTSDEDTMMAKTYTFKVPALPSTETKLCYACVRDGEIANSCGVMITVKPKGPTTEEIPSALLERGLCLPVYSTDVAKTGLRRPSVVLKVDKRNRVVEFTCPHSSLVFPDQAADSDAGEAVVYTVSGGSCDVWENPVYLTKILPGASLVSETAVDASEITTKYTFTVKQLPKTPKKLCYLCVYNRDVMNSCGVLIDVSSNSMTRLSKTSEEGIHTNPTVPTTLELQCPPDYSARTAATGLRLPEMELLVDSVNRTARFVCPDDSSVFPEIDGEADPASGKVYRMTGDSCDTREETAFLQDEVPGAELQRRTVVDGGVVQRYYIFKASRLPEEDKKLCFLCVRQRNPADSCAVMITVKADSAAAVPIHPFRPRPAVKLATYVCKPENSTEVAETGLKAPALSLTIDSRAHSIQFICPESSIVFPDLAAVPDQDSATVYLVGEGGSCNVAASPRLLSDVLPGATLGSRTTVDEGVVNRTYTLTAPKLPEEDVKLCYLCVRNRQIAESCGIHITVKGTKAESVAKPAGPICSLGYSPGSEKTGMREAAIELVVEDPSTPVRFICPEGSYVFPEYATSTDKGIAAVYGVKGNECIFAGPRENLQSLVPGATLRMEAADEGGTVMRTYTFTTPEQPAEDRRFCYMCVRERDIYQSCPVIIVVKGSGHLPEPKAQPQEEHELPVCTPHEQAGTALTGLLDPSVKLWVNEPEEQVSFVCPDGSAVLPDQETSEPQVYAVGAGEYCLVTKPLMSLAKAVPSASLSTDTVVENEVTTRKYTLRVPSLPLEETKLCYTCVSEVDPAKKCGVSVTVKGEGKMPGGLTSSLPSPVCAAQFSQCAFLTGVRMPSIMLTVHEPNTKLVFDCPPNTALYPQNAVVPGKATFFPLNEKGACIYKGPVAESKLYDVVPGARLRAKETVDGAVVRSYTLTVSKLPKKETRLCYLCVRGDEPAYSCGVIVKVKAPAPAAPEPKQLPVCVPSSDPSVGKMRRITPKLTLKIEKPGGSASFECPDGSTIFPDHADALDPKCVLAYKVVRDTCDLRGPTEMVASKLQGAYLTKTFVGTGYKYTFTVPHLPAEQQQVCFMCVMDRDTSRSCGVVINVMPHPAASRSSVPECKLKHVPAAATTGLREASLILNVREPSSVVEFGCPRNSVIMPSTATSSEHLAQVYSVRDRHICDMKEFLRPLADLVPGASLKLVHTPEDGDTTRTHMFRVGSLPVKDTALCYLCVDPGDHSHNCGVVINVKGSEVPPPPKDFGCAPSHSEEVERTGKLSPAVRLMVTSTKEPIRFECRDNAKVYPPAASLIKPAKAVVYPVSAGGRCIVGKPPLSLNRVVPGAKLKTKAKLVTGAITTTGFVFVPVLPSIQKDFCFACVDRGDITNSCGVLVTVPPFWAPPVQETVCNDVKTLTMTVHSPGSVTLRCGLEFPKVDPPIDDPASQGQVYYGKSCGDVGALRTVIPGASVVKEPFYHNLAKEVAVGVTLTVPASIVKQTICFKCRQPDPLQHETCTVRVTVLPPAAQPTTTTTTTTTTTIKPTTTTTTRKPTTTTTTTRRPTTTTTTTKKPTTTTTTTRKPRTTTTTTTKKPTTTTTTTRKPTTTTTTTKKPTTTTTTTKKPTTTTTTTKKPTTTTTTTTTRKPTTTTTTTKKPTTTTTTTKKPTTTTTTTTKKPTTTTTTTKKPTTTTTTTRKPTTTTTTTRKPTTTTTTNKPTTTTTTRTPTTTTSKPPVVFELPSEFIEETATTTRATISLRARSAAAPTSTTTVGPTTPATSLFDWSSKVASLAGQWSFSGALQGTAGSRSGVYEAPITQLPPPLLVPFKIDCCGPPVIQKGCCPPPLIQVDCCRPPVLQQKPGCCCCGHE